European Patent Specification EP 3 620 521 B1, published May 29, 2024. Title: GLOBIN GENE THERAPY FOR TREATING HEMOGLOBINOPATHIES. Applicant: MEMORIAL SLOAN-KETTERING CANCER CENTER. The sequence listing filed with the application follows.

SEQUENCE LISTING (26 sequences)

SEQ ID NO: 1 - DNA, 305 bp, Homo sapiens
tccttcctttctaaatgacgagagagacagaagaattcttcaaggttagtgtgtccagcatgcaacctttccttcctggatgagcatccctggagtaggagagccagcctgcctcctgcgctggcacagagcccggttccctagacaactgcctctccaaatctgatgtccagcgccacctggtgtccacatcaagcagacacaattaatagtcaacctgttcaggaaaactgtgagggggaaaaaaaagaaagaggatttatgaagggaaaagaaagtttagaggatatgccacgattggctag

SEQ ID NO: 2 - DNA, 1074 bp, Homo sapiens
aagtaaacttccacaaccgcaagcttattgaggctaaggcatctgtgaaggaaagaaacatctcctctaaaccactatgctgctagagcctcttttctgtactcaagcctcattcagacactagtgtcaccagtctcctcatatacctattgtattttcttcttcttgctggtttagtcatgttttctgggagcttaggggcttattttattttgttttgttttctaatcaacagagatgggcaaacccattatttttttctttagacttgggatggtgatagctgggcagcgtcagaaactgtgtgtggatatagataagagctcggactatgctgagctgtgatgagggagggacctagccaaaggcagtgagagtcagaatgctcctgctattgccttctcagtccccacgcttggtttctacacaagtagatacatagaaaaggctataggttagtgtttgagagtcctgcatgagttagttgctcagaaatgcccgataaatatgttatgtgtgtttatgtatatatatgttttatatatatatatgtgtgtgtgtgtgtgtgtgtgtgttgtgtttacaaatatgtgattatcatcaaaacgtgagggctaaagtgaccagataacttgcaggtcctaggataccaggaaaataaattacattccaaaaatttaactgagactttaaaaaaaaaaaaaaaaaaaaaaaaaaaaccagtgatccatggacacagggaggggaacatcacacactggggcctgttgggggtggggggctaggggaaggatagcattaggagaaatacctaatgtagatgacgggttgatgggtgcagcaaaccaccatggcacatgtaccccagaacttaaagcatattaaaaaaacagtgatcataaaagaagctcaaatttaactataagagacggaatggctcccacaattcttaactataatcttacagaatattctcattgaatagaagtatgcttatcattagagatttggacagccaggaaagcacagaaaaaaaaaaaaggagctctgttgccttatagcctagaggtgttt

SEQ ID NO: 3 - DNA, 602 bp, Homo sapiens
ggcatctgtgaaggaaagaaacatctcctctaaaccactatgctgctagagcctcttttctgtactcaagcctcattcagacactagtgtcaccagtctcctcatatacctattgtattttcttcttcttgctggtttagtcatgttttctgggagcttaggggcttattttattttgttttgttttctaatcaacagagatgggcaaacccattatttttttctttagacttgggatggtgatagctgggcagcgtcagaaactgtgtgtggatatagataagagctcggactatgctgagctgtgatgagggagggacctagccaaaggcagtgagagtcagaatgctcctgctattgccttctcagtccccacgcttggtttctacacaagtagatacatagaaaaggctataggttagtgtttgagagtcctgcatgagttagttgctcagaaatgcccgataaatatgttatgtgtgtttatgtatatatatgttttatatatatatatgtgtgtgtgtgtgtgtgtgtgtgttgtgtttacaaatatgtgattatcatcaaaacgtgagggctaaagtgaccagataacttgcagg

SEQ ID NO: 4 - DNA, 489 bp, Homo sapiens
ggcatctgtgaaggaaagaaacatctcctctaaaccactatgctgctagagcctcttttctgtactcaagcctcattcagacactagtgtcaccagtctcctcatatacctattgtattttcttcttcttgctggtttagtcatgttttctgggagcttaggggcttattttattttgttttgttttctaatcaacagagatgggcaaacccattatttttttctttagacttgggatggtgatagctgggcagcgtcagaaactgtgtgtggatatagataagagctcggactatgctgagctgtgatgagggagggacctagccaaaggcagtgagagtcagaatgctcctgctattgccttctcagtccccacgcttggtttctacacaagtagatacatagaaaaggctataggttagtgtttgagagtcctgcatgagttagttgctcagaaatgcccgataaatatgttatgtgtgtttatgt

SEQ ID NO: 5 - DNA, 1301 bp, Homo sapiens
aagctttcattaaaaaaagtctaaccagctgcattcgactttgactgcagcagctggttagaaggttctactggaggagggtcccagcccattgctaaattaacatcaggctctgagactggcagtatatctctaacagtggttgatgctatcttctggaacttgcctgctacattgagaccactgacccatacataggaagcccatagctctgtcctgaactgttaggccactggtccagagagtgtgcatctcctttgatcctcataataaccctatgagatagacacaattattactcttactttatagatgatgatcctgaaaacataggagtcaaggcacttgcccctagctgggggtataggggagcagtcccatgtagtagtagaatgaaaaatgctgctatgctgtgcctcccccacctttcccatgtctgccctctactcatggtctatctctcctggctcctgggagtcatggactccacccagcaccaccaacctgacctaaccacctatctgagcctgccagcctataacccatctgggccctgatagctggtggccagccctgaccccaccccaccctccctggaacctctgatagacacatctggcacaccagctcgcaaagtcaccgtgagggtcttgtgtttgctgagtcaaaattccttgaaatccaagtccttagagactcctgctcccaaatttacagtcatagacttcttcatggctgtctcctttatccacagaatgattcctttgcttcattgccccatccatctgatcctcctcatcagtgcagcacagggcccatgagcagtagctgcagagtctcacataggtctggcactgcctctgacatgtccgaccttaggcaaatgcttgactcttctgagctcagtcttgtcatggcaaaataaagataataatagtgtttttttatggagttagcgtgaggatggaaaacaatagcaaaattgattagactataaaaggtctcaacaaatagtagtagattttatcatccattaatccttccctctcctctcttactcatcccatcacgtatgcctcttaattttcccttacctataataagagttattcctcttattatattcttcttatagtgattctggatattaaagtgggaatgaggggcaggccactaacgaagaagatgtttctcaaagaagccattctccccacatagatcatctcagcagggttcaggaagataaaggaggatcaaggtcgaaggtaggaactaaggaagaacactgggcaagtggatcc

SEQ ID NO: 6 - DNA, 1065 bp, Homo sapiens
tgagccccttttcctctaactgaaagaaggaaaaaaaaaatggaacccaaaatattctacatagtttccatgtcacagccagggctgggcagtctcctgttatttcttttaaaataaatatatcatttaaatgcataaataagcaaaccctgctcgggaatgggagggagagtctctggagtccaccccttctcggccctggctctgcagatagtgctatcaaagccctgacagagccctgcccattgctgggccttggagtgagtcagcctagtagagaggcagggcaagccatctcatagctgctgagtgggagagagaaaagggctcattgtctataaactcaggtcatggctattcttattctcacactaagaaaaagaatgagatgtctacatataccctgcgtcccctcttgtgtactggggcccccaagagctctctaaaagtgatggcaaagtcattgcgctagatgccatcccatctattataaacctgcatttgtctccacacaccagtcatggacaataaccctcctcccaggtccacgtgcttgtctttgtataatactcaagtaatttcggaaaatgtattctttcaatcttgttctgttattcctgtttcaatggcttagtagaaaaagtacatacttgttttcccataaattgacaatagacaatttcacatcaatgtctatatgggtcgttgtgtttgctgtgtttgcaaaaactcacaataactttatattgttactactctaagaaagttacaacatggtgaatacaagagaaagctattacaagtccagaaaataaaagttatcatcttgaggcctcagctttctaggaataatatcaatattacaaaatttaatctaacaattatgaacagcaatgagataatatgtacaaagtacccagacctatgtggtagagcatcaaggaagcgcattgcggagcagttttttgtttgtttgtttttgtattctgtttcgtgaggcaaggtttcactctgctgtccaggctggagtgcagtggcaagatcatgtctcactgcagccttgac

SEQ ID NO: 7 - DNA, 1065 bp, Homo sapiens
tgagccccttttcctctaactgaaagaaggaaaaaaaaaatggaacccaaaatattctacatagtttccatgtcacagccagggctgggcagtctcctgttatttcttttaaaataaatatatcattaaatgcataaataagcaaaccctgctcgggaatgggagggagagtctctggagtccaccccttctcggccctggctctgcagatagtgctatcaaagccctgacagagccctgcccattgctgggccttggagtgagtcagcctagtagagaggcagggcaagccatctcatagctgctgagtgggagagagaaaagggctcattgtctataaactcaggtcatggctattcttattctcacactaagaaaaagaatgagatgtctacatataccctgcgtcccctcttgtgtactggggcccccaagagctctctaaaagtgatggcaaagtcattgcgctagatgccatcccatctattataaacctgcatttgtctccacacaccagtcatggacaataaccctcctcccaggtccacgtgcttgtctttgtataatactcaagtaatttcggaaaatgtattctttcaatcttgttctgttattcctgtttcaatggcttagtagaaaaagtacatacttgttttcccataaattgacaatagacaatttcacatcaatgtctatatgggtcgttgtgtttgctgtgtttgcaaaaactcacaataactttatattgttactactctaagaaagttacaacatggtgaatacaagagaaagctattacaagtccagaaaataaaagttatcatcttgaggcctcagctttctaggaataatatcaatattacaaaattaatctaacaattatgaacagcaatgagataatatgtacaaagtacccagacctatgtggtagagcatcaaggaagcgcattgcggagcagttttttgtttgtttgtttttgtattctgtttcgtgaggcaaggtttcactctgctgtccaggctggagtgcagtggcaagatcatgtctcactgcagccttgacac

SEQ ID NO: 8 - DNA, 446 bp, Homo sapiens
tggaacccaaaatattctacatagtttccatgtcacagccagggctgggcagtctcctgttatttcttttaaaataaatatatcatttaaatgcataaataagcaaaccctgctcgggaatgggagggagagtctctggagtccaccccttctcggccctggctctgcagatagtgctatcaaagccctgacagagccctgcccattgctgggccttggagtgagtcagcctagtagagaggcagggcaagccatctcatagctgctgagtgggagagagaaaagggctcattgtctataaactcaggtcatggctattcttattctcacactaagaaaaagaatgagatgtctacatataccctgcgtcccctcttgtgtactggggtccccaagagctctctaaaagtgatggcaaagtcattgcgctagatgccatcccatct

SEQ ID NO: 9 - DNA, 860 bp, Homo sapiens
gtatatgtgtatatatatatatatatattcaggaaataatatattctagaatatgtcacattctgtctcaggcatccattttctttatgatgccgtttgaggtggagttttagtcaggtggtcagcttctccttttttttgccatctgccctgtaagcatcctgctggggacccagataggagtcatcactctaggctgagaacatctgggcacacaccctaagcctcagcatgactcatcatgactcagcattgctgtgcttgagccagaaggtttgcttagaaggttacacagaaccagaaggcgggggtggggcactgaccccgacaggggcctggccagaactgctcatgcttggactatgggaggtcactaatggagacacacagaaatgtaacaggaactaaggaaaaactgaagcttatttaatcagagatgagatgctggaagggatagagggagctgagcttgtaaaaagtatagtaatcattcagcaaatggttttgaagcacctgctggatgctaaacactattttcagtgcttgaatcataaataagaataaaacatgtatcttattccccacaagagtccaagtaaaaaataacagttaattataatgtgctctgtcccccaggctggagtgcagtggcacgatctcagctcactgcaacctccgcctcccgggttcaagcaattctcctgcctcagccaccctaatagctgggattacaggtgcacaccaccatgccaggctaatttttgtactttttgtagaggcagggtatcaccatgttgtccaagatggtcttgaactcctgagctccaagcagtccacccacctcagcctcccaaagtgct

SEQ ID NO: 10 - DNA, 613 bp, Homo sapiens
aagcaatagatggctctgccctgacttttatgcccagccctggctcctgccctccctgctcctgggagtagattggccaaccctagggtgtggctccacagggtgaggtctaagtgatgacagccgtacctgtccttggctcttctggcactggcttaggagttggacttcaaaccctcagccctccctctaagatatatctcttggccccataccatcagtacaaattgctactaaaaacatcctcctttgcaagtgtatttacgtaatatttggaatcacagcttggtaagcatattgaagatcgttttcccaattttcttattacacaaataagaaattgatgcactaaaagtggaagagttttgtctaccataattcagctttgggatatgtagatggatctcttcctgcgtctccagaatatgcaaaatacttacaggacagaatggatgaaaactctacctcagttctaagcatatcttctccttatttggattaaaaccttctggtaagaaaagaaaaaaaatatatatatatatgtgtatatatacacacatacatatacatatatatgcattcatttgttgttgtttttcttaatttgctcatg

SEQ ID NO: 11 - DNA, 265 bp, Homo sapiens
aagcaatagatggctctgccctgacttttatgcccagccctggctcctgccctccctgctcctgggagtagattggccaaccctagggtgtggctccacagggtgaggtctaagtgatgacagccgtacctgtccttggctcttctggcactggcttaggagttggacttcaaaccctcagccctccctctaagatatatctcttggccccataccatcagtacaaattgctactaaaaacatcctcctttgcaagtgtatttac

SEQ ID NO: 12 - DNA, 879 bp, Homo sapiens
taggtattgaataagaaaaatgaagttaaggtggttgatggtaacactatgctaataactgcagagccagaagcaccataagggacatgataagggagccagcagacctctgatctcttcctgaatgctaatcttaaacatcctgaggaagaatgggacttccatttggggtgggcctatgatagggtaataagacagtagtgaatatcaagctacaaaaagccccctttcaaattcttctcagtcctaacttttcatactaagcccagtccttccaaagcagactgtgaaagagtgatagttccgggagactagcactgcagattccgggtcactgtgagtgggggaggcagggaagaagggctcacaggacagtcaaaccatgccccctgtttttccttcttcaagtagacctctataagacaacagagacaactaaggctgagtggccaggcgaggagaaaccatctcgccgtaaaacatggaaggaacacttcaggggaaaggtggtatctctaagcaagagaactgagtggagtcaaggctgagagatgcaggataagcaaatgggtagtgaaaagacattcatgaggacagctaaaacaataagtaatgtaaaatacagcatagcaaaactttaacctccaaatcaagcctctacttgaatccttttctgagggatgaataaggcataggcatcaggggctgttgccaatgtgcattagctgtttgcagcctcaccttctttcatggagtttaagatatagtgtattttcccaaggtttgaactagctcttcatttctttatgttttaaatgcactgacctcccacattccctttttagtaaaatattcagaaataatttaaatacatcattg

SEQ ID NO: 13 - DNA, 152 bp, Artificial Sequence
  Description of Artificial Sequence: Synthetic polynucleotide
tctcccacgccctggtctcagcttggggagtggtcagaccccaatggcgataaactctggcaactttatctgtgcactgcaggctcagccccaacagctttagctttcacaagcaggcaggggaagggaaacacatatctccagatatgagg

SEQ ID NO: 14 - DNA, 157 bp, Artificial Sequence
  Description of Artificial Sequence: Synthetic polynucleotide
ctaaacccctcccccaccctagccccaagcttcatcttagctccactcctgaccctatccagctaaaggtccccacccagctcctgcctatctagtcattgcatatggcaagacttgaaagtcctatctcaaagcagcagaattatcagctacgact

SEQ ID NO: 15 - DNA, 141 bp, Artificial Sequence
  Description of Artificial Sequence: Synthetic polynucleotide
ccatcccccagcactccctgcccccacagcccagacttgaccaactcccagctccgcctgggacttccagatatggggccccacccttgcaggccttggggacgctgaagatattgactatctgcgtgccggaaaagggtg

SEQ ID NO: 16 - DNA, 171 bp, Artificial Sequence
  Description of Artificial Sequence: Synthetic polynucleotide
aaaggctgggggtgggagtagcggatttgaagcacttgttggcctacagaggtgtggcaagcagagcacctcagaactcaggcgtactgcccgccgcccgagccctgcgagggccgatagcgagggtgtggcccttatctgcacccagcagagcgccggcggggtacggtc

SEQ ID NO: 17 - DNA, 195 bp, Artificial Sequence
  Description of Artificial Sequence: Synthetic polynucleotide
cagttgcctcagctgagtatgtcttctaaagataatgtcgattgtgtatggctgatgggattctaggaccaagcaagaggtttttttttttcccccacatacttaacgtttctatatttctatttgaattcgactggacagttccatttgaattatttctctctctctctctctctgacacattttatcttgcca

SEQ ID NO: 18 - DNA, 14 bp, Homo sapiens
caccaggtggcgct

SEQ ID NO: 19 - DNA, 81706 bp, Homo sapiens
ggatcctcacatgagttcagtatataattgtaacagaataaaaaatcaattatgtattcaagttgctagtgtcttaagaggttcacatttttatctaactgattatcacaaaaatacttcgagttacttttcattataattcctgactacacatgaagagactgacacgtaggtgccttacttaggtaggttaagtaatttatccaaaaccacacaatgtagaacctaagctgattcggccatagaaacacaatatgtggtataaatgagacagagggatttctctccttcctatgctgtcagatgaatactgagatagaatatttagttcatctatcacacattaaacgggactttacatttctgtctgttgaagatttgggtgtggggataactcaaggtatcatatccaagggatggatgaaggcaggtgactctaacagaaagggaaaggatgttggcaaggctatgttcatgaaagtatatgtaaaatccacattaagcttctttctgcatgcattggcaatgtttatgaataatgtgtatgtaaaagtgtgctgtatattcaaaagtgtttcatgtgcctaggggtgtcaaatactttgagtttgtaagtatatacttctctgtaatgtgtctgaatatctctatttacttgattctcaataagtaggtatcatagtgaacatctgacaaatgtttgaggaacaatttagtgtttacctattcaccaaaatttattaaatgcctaatctgtatcagatatacaattatctggcgaaatctgtaattcctaatttaaacagctgtgtagcctaattagggataaaggcatgcaaacccataatttgtgtaggttgaaatgagctatagaaaaatgcagtatatttatcagaagtctttagggtcatgaaaaggaatggtcaactgacactgccagggactcatatgtaagagataactaatgtgaagtgactttaaaggagaaattagcagaagttttctttccatgtctcctcatcatgttacaataacggaagagattaaaacaacaaatacatttagacagcaatgtttatcctggttagatgttttaatctaaatctatcttggagtgttaaaatgcatttgctcacctactttaaaatataaatgaaggtaggaacctgtagatacaaaaagttggagaaaaaaagacaataaagatgacaaaaatctattaatccttgatagaaaatgagaagagataaaacactggtttacataaagaaaataagatggatagatagcagatccttataaaagtgataatttgagaaaaaaaatactccatattctgagtttcttcacataaaataatacaaatctgctgtggtaagttacaaagagatagattttttatcattatataaaagatattttaaacagagttatacaacaaaggaacagactatgtcatatattctcacttatcactataaacatctcagaaaaatctgcaaaatcatttcatagcattttaaatagttaggaataatgtagaaaactgaaacagttctaagtttcccacaaacttagagtctcaaatgttgcattacctaacttacctgcaaatattttatacaaatttgcacatgctactctagtcaaaaatatatgtacattatgggtattttctgtgtgtaacttggttctagttgcttctttcagaaatagcctctatttttgatttacctgataaaatcacattcctctccaaagccttctaaatacttccagactaactactttttagtacatctaagaagaaaagagttttgtctcttatccacctctgagtcaaaaagcagcatgtccatcaattggtacatagttcccacagccccacttagctctggattggagttctacttggcattgtttgcaactacatggacgtaaaatgcatggattctcttgaaaaaatgtttctgccatgatgttctctgaaagagactaaccttccctcgctttgcagagaaagactcgtgtaatccttgacaatgtcatctcatctatttattcccatgtctacccatatgtgaccttcatgtctttgctctaagcccctacatcctcaatctacacactaggatagtataaaagtaatagtaataatagtagtaatagtaataacaatacaatgattatggcttatactatacacaagacactgttgatatattatttcatttagtattcacagtaactctgtgcctcaagtactattgtaataccctttaagaggaggaaactgaggcacagggccctaaagtaatattccaagatgaagtggctactaactgacagagggcataattcaactcatgatatttggctctagaatacatgctctgaatcattatacaataataattcatgaggaaacattttttaaagcctaagttatttgctctgaaataagacataatttggggtgagaaagcttagattccatgaagtattacagcatttggtagtctttttgcactccaggtcttatttttactgcttaaacataataaaacatatggttcagtatgcctttgattttacaataatattcctgttatttttggaagcacagggtgtgggataatgctaattactagtgattagtattgagaggtgacagcgtgctggcagtcctcacagccctcgctcgctcttggcgcctcctctgcctgggctcccacattggtggcacttgaggagcccttcagccggccgctgcactgtgggagcccttttctgggctggccaaggccagagccggctccctcagcttgccaggaggtgtggagggacagacgcgggcaggaaccgggctgtgcgccgtgcttgagggagttccgggtgggcatgggctccgaggaccccgcactcggagccgccagccggccccaccggccgcgggcagtgaggggcttagcacctgggccagcagctgctgtgctcaattcctcgccgggccttagctgccttcctgcggggcagggctcgggacctgcagcgcgccatgcctgagcctccccaccttcatgggctcctgtgcggcccgagcctcgccgacgagcgccgccccctgctccagggcacccagtcccatcgaccacccaagggctgaagagtgcgggcgcacggcaggggactggcaggcagctccccctgcagcccaggtgcgggatccactgggtgaagccggctaggctcctgagtttgctggggatgcgaagaacccttatgtctagataagggattgtaaatacaccaattggcactctgtatctagctcaaggtttgtaaacacaccaatcagcaccctgtgtctagctcagggtttgtgaatgcaccaatcaacactctatctagctactctggtggggccttggagaacctttatgtctagctcagggattgtaaatacaccaatcggcagtctgtatctagctcaaggtttgtaaacacaccaatcagcaccctgtgtctagctcagggtttgtgaatgcaccaatcaacactctgtatctagctactctggtggggacgtggagaacctttatgtctagctcagggattgtaaatacaccactcggcagtctgtatctagctcaaggtttgtaaacacaccaatcagcaccctgtgtctagctcagggtttgtgaatgcaccaatcaacactctgtatctagctactctggtggggacttggagaacctttgtgtggacactctgtatctagctaatctggtggggacgtggagaacctttgtgtctagctcatggattgtaaatgcaccaatcagtgccctgtcaaaacagaccactgggctctaccaatcagcaggatgtgggtggggccagataagagaataaaagcaggctgcccgagccagcagtggcaacccgctcgggtccccttccacactgtggaagctttgttctttcgctctttgcaataaatcttgctgctgctcactgtttgggtctacactgcctttatgagctgtaacgctcaccgcgaaggtctgcagcttcactcttgaagccagcgagaccacgaacccaccgggaggaacgaacaactccagaggcgccgccttaagagctggaacgttcactgtgaaggtctgcagcttcactcctgagccagcgagaccacgaacccatcagaaggaagaaactccgaacacatccaaacatcagaacgaacaaactccacacacgcagcctttaagaactgtaacactcaccacgagggtccccggcttcattcttgaagtcagtgaaaccaagaacccaccaattccggacacagtatgtcagaaacaatatgagtcactaaatcaatatacttctcaacaatttccaacagcccttgcaattaacttggccatgtgactggttgtgactaaaataatgtggagataataatgtgttactccctaaggcagagtgcccttctatcattctctttcccttcctctatgtggcagaaagtaaaagattctgaaatgataaagtcaatcacaggaaggcacctggactcctggcccactgcttggaggagagcactcaggaccatgaacatctgactgtgacgtagcaataaagaaacccacgtttcatatgaaactgcttaaaattaatggcacaagtcatgtttttgatgttgcacatttgtctttatttgtggcttgttttgcttccacatcaatccactcaaggcctacattctgctataatgcaatttcaagttctttacaggccgagaaaaatgaatctgaattcctgacctccaaaagtgatcaagatatttttagttcaggctccaaaattttctcattttcataggttttcctcgattgatcattattcatgatttgcaaggaatcattcaatgttttctaaatctattactgcatcctgacacatatgacattttaactatgttccagatttttgaatgaagagtgtaaattttaaatgttttcaccacaaaaaataagtatgtgaagtggtggatttgttaattagccttatttaaccatttaatattgtacacgtacaccaaagcatcatgttgtaccccatgaatacacacaattattatttgtcaatttaaaatgaaataataaaaaataacaaaggcattagcctctgcattgcctttaccggtcatcctcacggtgactaacgcaaaaaacgttctatttcatccttacaaacatccctatctttgatgcctctttgtctagatctctatcccctcctgttttctctacgttatttatatgggtatcatcaccatcctggacaacatcaggacagatatccctcaccaagccaatgttcctctctatgttggctcaaatgtccttgaactttcctttcaccaccctttccacagtcaaaaggatattgtagtttaatgcctcagagttcagcttttaagcttctgacaaattattcttcctctttaggttctcctttatggaatcttctgtactgatggccatgtcctttaactactatgtagatatctgctactacctgtattatgcctctacctttattagcagagttatctgtactgttggcatgacaatcatttgttaatatgacttgcctttcctttttctgctattcttgatcaaatggctcctctttcttgctcctctcatttctcctgccttcacttggacgtgcttcacgtagtctgtgcttatgactggattaaaaattgatatggacttatcctaatgttgttcgtcataatatgggttttatggtccattattatttcctatgcattgatctggagaaggcttcaatccttttactctttgtggaaaatatctgtaaaccttctggttcactctgctatagcaatttcagtttaggctagtaagcatgaggatgcctccttctctgatttttcccacagtctgttggtcacagaataacctgagtgattactgatgaaagagtgagaatgttattgatagtcacaatgacaaaaaacaaacaactacagtcaaaatgtttctctttttattagtggattatatttcctgacctatatctggcaggactctttagagaggtagctgaagctgctgttatgaccactagagggaagaagatacctgtggagctaatggtccaagatggtggagccccaagcaaggaagttgttaaggagcccttttgattgaaggtgggtgcccccaccttacagggacaggacatctggatactcctcccagtttctccagtttccctttttcctaatatatctcctgataaaatgtctatactcacttccccatttctaataataaagcaaaggctagttagtaagacatcaccttgcattttgaaaatgccatagactttcaaaattatttcatacatcggtctttctttatttcaagagtccagaaatggcaacattacctttgattcaatgtaatggaaagagctctttcaagagacagagaaaagaataatttaatttctttccccacacctccttccctgtctcttaccctatcttccttccttctaccctccccatttctctctctcatttctcagaagtatattttgaaaggattcatagcagacagctaaggctggttttttctaagtgaagaagtgatattgagaaggtagggttgcatgagccctttcagttttttagtttatatacatctgtattgttagaatgttttataatataaataaaattatttctcagttatatactagctatgtaacctgtggatatttccttaagtattacaagctatacttaactcacttggaaaactcaaataaatacctgcttcatagttattaataaggattaagtgagataatgcccataagattcctattaataacagataaatacatacacacacacacacattgaaaggattcttactttgtgctaggaactataataagttcattgatgcattatatcattaagttctaatttcaacactagaaggcaggtattatctaaatttcatactggatacctccaaactcataaagataattaaattgccttttgtcatatatttattcaaaagggtaaactcaaactatggcttgtctaattttatatatcaccctactgaacatgaccctattgtgatattttataaaattattctcaagttattatgaggatgttgaaagacagagaggatggggtgctatgccccaaatcagcctcacaattaagctaagcagctaagagtcttgcagggtagtgtagggaccacagggttaagggggcagtagaattatactcccactttagtttcatttcaaacaatccatacacacacagccctgagcacttacaaattatactacgctctatactttttgtttaaatgtataaataagtggatgaaagaatagatagatagatagacagatagatgatagatagaataaatgcttgccttcatagctgtctccctaccttgttcaaaatgttcctgtccagaccaaagtaccttgccttcacttaagtaatcaattcctaggttatattctgatgtcaaaggaagtcaaaagatgtgaaaaacaatttctgacccacaactcatgctttgtagatgactagatcaaaaaatttcagccatatcttaacagtgagtgaacaggaaatctcctcttttccctacatctgagatcccagcttctaagaccttcaattctcactcttgatgcaacagaccttggaagcatacaggagagctgaacttggtcaacaaaggagaaaagtttgttggcctccaaaggcacagctcaaacttttcaagccttctctaatcttaaaggtaaacaagggtctcatttctttgagaacttcagggaaaatagacaaggacttgcctggtgcttttggtaggggagcttgcactttccccctttctggaggaaatatttatccccaggtagttccctttttgcaccagtggttctttgaagagacttccacctgggaacagttaaacagcaactacagggccttgaactgcacactttcagtccggtcctcacagttgaaaagacctaagcttgtgcctgatttaagcctttttggtcataaaacattgaattctaatctccctctcaaccctacagtcacccatttggtatattaaagatgtgttgtctactgtctagtatccctcaagtagtgtcaggaattagtcatttaaatagtctgcaagccaggagtggtggctcatgtctgtaattccagcacttgagaggtagaagtgggaggactgcttgagctcaagagtttgatattatcctggacaacatagcaagacctcgtctctacttaaaaaaaaaaaaaaaattagccaggcatgtgatgtacacctgtagtcccagctactcaggaggccgaaatgggaggatcccttgagctcaggaggtcaaggctgcagtgagacatgatcttgccactgcactccagcctggacagcagagtgaaaccttgcctcacgaaacagaatacaaaaacaaacaaacaaaaaactgctccgcaatgcgcttccttgatgctctaccacataggtctgggtactttgtacacattatctcattgctgttcataattgttagattaattttgtaatattgatattattcctagaaagctgaggcctcaagatgataacttttattttctggacttgtaatagctttctcttgtattcaccatgttgtaactttcttagagtagtaacaatataaagttattgtgagtttttgcaaacacagcaaacacaacgacccatatagacattgatgtgaaattgtctattgtcaatttatgggaaaacaagtatgtactttttctactaagccattgaaacaggaataacagaacaagattgaaagaatacattttccgaaattacttgagtattatacaaagacaagcacgtggacctgggaggagggttattgtccatgactggtgtgtggagacaaatgcaggtttataatagatgggatggcatctagcgcaatgactttgccatcacttttagagagctcttggggaccccagtacacaagaggggacgcagggtatatgtagacatctcattctttttcttagtgtgagaataagaatagccatgacctgagtttatagacaatgagcccttttctctctcccactcagcagctatgagatggcttgccctgcctctctactaggctgactcactccaaggcccagcaatgggcagggctctgtcagggctttgatagcactatctgcagagccagggccgagaaggggtggactccagagactctccctcccattcccgagcagggtttgcttatttatgcatttaaatgatatatttattttaaaagaaataacaggagactgcccagccctggctgtgacatggaaactatgtagaatattttgggttccatttttttttccttctttcagttagaggaaaaggggctcactgcacatacactagacagaaagtcaggagctttgaatccaagcctgatcatttccatgtcatactgagaaagtccccacccttctctgagcctcagtttctctttttataagtaggagtctggagtaaatgatttccaatggctctcatttcaatacaaaatttccgtttattaaatgcatgagcttctgttactccaagactgagaaggaaattgaacctgagactcattgactggcaagatgtccccagaggctctcattcagcaataaaattctcaccttcacccaggcccactgagtgtcagatttgcatgcactagttcacgtgtgtaaaaaggaggatgcttctttcctttgtattctcacatacctttaggaaagaacttagcacccttcccacacagccatcccaataactcatttcagtgactcaacccttgactttataaaagtcttgggcagtatagagcagagattaagagtacagatgctggagccagaccacctgagtgattagtgactcagtttctcttagtagttgtatgactcagtttcttcatctgtaaaatggagggttttttaattagtttgtttttgagaaagggtctcactctgtcacccaaatgggagtgtagtggcaaaatctcggctcactgcaacttgcacttcccaggctcaagcggtcctcccacctcaacatcctgagtagctggaaccacaggtacacaccaccatacctcgctaattttttgtatttttggtagagatggggtttcacatgttacacaggatggtctcagactccggagctcaagcaatctgcccacctcagccttccaaagtgctgggattataagcatgattacaggagttttaacaggctcataagattgttctgcagcccgagtgagttaatacatgcaaagagtttaaagcagtgacttataaatgctaactactctagaaatgtttgctagtattttttgtttaactgcaatcattcttgctgcaggtgaaaactagtgttctgtactttatgcccattcatctttaactgtaataataaaaataactgacatttattgaaggctatcagagactgtaattagtgctttgcataattaatcatatttaatactcttggattctttcaggtagatactattattatccccattttactacagttaaaaaaactacctctcaacttgctcaagcatacactctcacacacacaaacataaactactagcaaatagtagaattgagatttggtcctaattatgtctttgctcactatccaataaatatttattgacatgtacttcttggcagtctgtatgctggatgctggggatacaaagatgtttaaatttaagctccagtctctgcttccaaaggcctcccaggccaagttatccattcagaaagcattttttactctttgcattccactgtttttcctaagtgactaaaaaattacactttattcgtctgtgtcctgctctgggatgatagtctgactttcctaacctgagcctaacatccctgacatcaggaaagactacaccatgtggagaaggggtggtggttttgattgctgctgtcttcagttagatggttaactttgtgaagttgaaaactgtggctctctggttgactgttagagttctggcacttgtcactatgcctattatttaacaaatgcatgaatgcttcagaatatgggaatattatcttctggaatagggaatcaagttatattatgtaacccaggattagaagattcttctgtgtgtaagaatttcataaacattaagctgtctagcaaaagcaagggcttggaaaatctgtgagctcctcaccatatagaaagcttttaacccatcattgaataaatccctataggggatttctaccctgagcaaaaggctggtcttgattaattcccaaactcatatagctctgagaaagtctatgctgttaacgttttcttgtctgctaccccatcatatgcacaacaataaatgcaggcctaggcatgactgaaggctctctcataattcttggttgcatgaatcagattatcaacagaaatgttgagacaaactatggggaagcagggtatgaaagagctctgaatgaaatggaaaccgcaatgcttcctgcccattcagggctccagcatgtagaaatctggggctttgtgaagactggcttaaaatcagaagccccattggataagagtagggaagaacctagagcctacgctgagcaggtttccttcatgtgacagggagcctcctgccccgaacttccagggatcctctcttaagtgtttcctgctggaatctcctcacttctatctggaaatggtttctccacagtccagcccctggctagttgaaagagttacccatgcagaggccctcctagcatccagagactagtgcttagattcctactttcagcgttggacaacctggatccacttgcccagtgttcttccttagttcctaccttcgaccttgatcctcctttatcttcctgaaccctgctgagatgatctatgtggggagaatggcttctttgagaaacatcttcttcgttagtggcctgcccctcattcccactttaatatccagaatcactataagaagaatataataagaggaataactcttattataggtaagggaaaattaagaggcatacgtgatgggatgagtaagagaggagagggaaggattaatggacgataaaatctactactatttgttgagaccttttatagtctaatcaattttgctattgttttccatcctcacgctaactccataaaaaaacactattattatctttattttgccatgacaagactgagctcagaagagtcaagcatttgcctaaggtcggacatgtcagaggcagtgccagacctatgtgagactctgcagctactgctcatgggccctgtgctgcactgatgaggaggatcagatggatggggcaatgaagcaaaggaatcattctgtggataaaggagacagccatgaagaagtctatgactgtaaatttgggagcaggagtctctaaggacttggatttcaaggaattttgactcagcaaacacaagaccctcacggtgactttgcgagctggtgtgccagatgtgtctatcagaggttccagggagggtggggtggggtcagggctggccaccagctatcagggcccagatgggttataggctggcaggctcagataggtggttaggtcaggttggtggtgctgggtggagtccatgactcccaggagccaggagagatagaccatgagtagagggcagacatgggaaaggtgggggaggcacagcatagcagcatttttcattctactactacatgggactgctcccctatacccccagctaggggcaagtgccttgactcctatgttttcaggatcatcatctataaagtaagagtaataattgtgtctatctcatagggttattatgaggatcaaaggagatgcacactctctggaccagtggcctaacagttcaggacagagctatgggcttcctatgtatgggtcagtggtctcaatgtagcaggcaagttccagaagatagcatcaaccactgttagagatatactgccagtctcagagcctgatgttaatttagcaatgggctgggaccctcctccagtagaaccttctaaccagctgctgcagtcaaagtcgaatgcagctggttagactttttttaatgaaagcttagctttcattaaagattaagctcctaagcagggcacagatgaaattgtctaacagcaactttgccatctaaaaaaatctgacttcactggaaacatggaagcccaaggttctgaacatgagaaatttttaggaatctgcacaggagttgagagggaaacaagatggtgaagggactagaaaccacatgagagacacgaggaaatagtgtagatttaggctggaggtaaatgaaagagaagtgggaattaatacttactgaaatctttctatatgtcaggtgccattttatgatatttaataatctcattacatatggtaattctgtgagatatgtattattgaacatactataattaatactaatgataagtaacacctcttgagtacttagtatatgctagaatcaaatttaagtttatcatatgaggccgggcacggtggctcatatatgggattacatgcctgtaatcccagcactttgggaggccaaggcaattggatcacctgaggtcaggagttccagaccagcctggccaacatggtgaaaccccttctctactaaaaaatacaaaaaatcagccaggtgtggtggcacgcgtctataatcccagctactcaggaggctgaggcaggagaatcacttgaacccaggaggtggaggttgcagtgagctaagattgcaccactgcactccagcctaggcgacagagtgagactccatctcaaaaaaaaaaaaagaagtttattatatgaattaacttagttttactcacaccaatactcagaagtagattattacctcatttattgatgaggagcccaatgtacttgtagtgtagatcaacttattgaaagcacaagctaataagtagacaattagtaattagaagtcagatggtctgagctctcctactgtctacattacatgagctcttattaactggggactcgaaaatcaaagacatgaaataatttgtccaagcttacagaaccaccaagtagtaaggctaggatgtagacccagttctgctacctctgaagacagtgttttttccacagcaaaacacaaactcagatattgtggatgcgagaaattagaagtagatattcctgccctgtggcccttgcttcttacttttacttcttgtcgattggaagttgtggtccaagccacagttgcagaccatacttcctcaaccataattgcatttcttcaggaaagtttgagggagaaaaaggtaaagaaaaatttagaaacaacttcagaataaagagattttctcttgggttacagagattgtcatatgacaaattataagcagacacttgagaaaactgaaggcccatgcctgcccaaattaccctttgaccccttggtcaagctgcaactttggttaaagggagtgtttatgtgttatagtgttcatttactcttctggtctaacccattggctccgtcttcatcctgcagtgacctcagtgcctcagaaacatacatatgtttgtctagtttaagtttgtgtgaaattctaactagcgtcaagaactgagggccctaaactatgctaggaatagtgctgtggtgctgtgataggtacacaagaaatgagaagaaactgcagattctctgcatctccctttgccgggtctgacaacaaagtttccccaaattttaccaatgcaagccatttctccatatgctaactactttaaaatcatttggggcttcacattgtctttctcatctgtaaaaagaatggaagaactcattcctacagaactccctatgtcttccctgatgggctagagttcctctttctcaaaaattagccattattgtatttccttctaagccaaagctcagaggtcttgtattgcccagtgacatgcacactggtcaaaagtaggctaagtagaagggtactttcacaggaacagagagcaaaagaggtgggtgaatgagagggtaagtgagaaaagacaaatgagaagttacaacatgatggcttgttgtctaaatatctcctagggaattattgtgagaggtctgaatagtgttgtaaaataagctgaatctgctgccaacattaacagtcaagaaatacctccgaataactgtacctccaattattctttaaggtagcatgcaactgtaatagttgcatgtatatatttatcataatactgtaacagaaaacacttactgaatatatactgtgtccctagttctttacacaataaactaatctcatcctcataattctattagctaatacatattatcatcctatatttcagagacttcaagaagttaagcaacttgctcaagatcatctaagaagtaggtggtatttctgggctcatttggcccctcctaatctctcatggcaacatggctgcctaaagtgttgattgccttaattcatcagggatgggctcatactcactgcagaccttaactggcatcctcttttcttatgtgatctgcctgaccctagtagacttatgaaatttctgatgagaaaggagagaggagaaaggcagagctgactgtgatgagtgatgaaggtgccttctcatctgggtaccagtggggcctctaagactaagtcactctgtctcactgtgtcttagccagttccttacagcttgccctgatgggagatagagaatgggtatcctccaacaaaaaaataaattttcatttctcaaggtccaacttatgttttcttaatttttaaaaaaatcttgaccattctccactctctaaaataatccacagtgagagaaacattcttttcccccatcccataaatacctctattaaatatggaaaatctgggcatggtgtctcacacctgtaatcccagcactttgggaggctgaggtgggtggactgcttggagctcaggagttcaagaccatcttggacaacatggtgataccctgcctctacaaaaagtacaaaaattagcctggcatggtggtgtgcacctgtaatcccagctattagggtggctgaggcaggagaattgcttgaacccgggaggcggaggttgcagtgagctgagatcgtgccactgcactccagcctgggggacagagcacattataattaactgttattttttacttggactcttgtggggaataagatacatgttttattcttatttatgattcaagcactgaaaatagtgtttagcatccagcaggtgcttcaaaaccatttgctgaatgattactatactttttacaagctcagctccctctatcccttccagcatcctcatctctgattaaataagcttcagtttttccttagttcctgttacatttctgtgtgtctccattagtgacctcccatagtccaagcatgagcagttctggccaggcccctgtcggggtcagtgccccacccccgccttctggttctgtgtaaccttctaagcaaaccttctggctcaagcacagcaatgctgagtcatgatgagtcatgctgaggcttagggtgtgtgcccagatgttctcagcctagagtgatgactcctatctgggtccccagcaggatgcttacagggcagatggcaaaaaaaaggagaagctgaccacctgactaaaactccacctcaaacggcatcataaagaaaatggatgcctgagacagaatgtgacatattctagaatatattatttcctgaatatatatatatatatacacatatacgtatatatatatatatatatatatttgttgttatcaattgccatagaatgattagttattgtgaatcaaatatttatcttgcaggtggcctctatacctagaagcggcagaatcaggctttattaatacatgtgtatagatttttaggatctatacacatgtattaatatgaaacaaggatatggaagaggaaggcatgaaaacaggaaaagaaaacaaaccttgtttgccattttaaggcacccctggacagctaggtggcaaaaggcctgtgctgttagaggacacatgctcacatacggggtcagatctgacttggggtgctactgggaagctctcatcttaaggatacatctcaggccagtcttggtgcattaggaagatgtaggcaactctgatcctgagaggaaagaaacattcctccaggagagctaaaagggttcacctgtgtgggtaactgtgaaggactacaagaggatgaaaaacaatgacagacagacataatgcttgtgggagaaaaaacaggaggtcaaggggatagagaaggcttccagaagaatggctttgaagctggcttctgtaggagttcacagtggcaaagatgtttcagaaatgtgacatgacttaaggaactatacaaaaaggaacaaatttaaggagaggcagataaattagttcaacagacatgcaaggaattttcagatgaatgttatgtctccactgagcttcttgaggttagcagctgtgagggttttgcaggcccaggacccattacaggacctcacgtatacttgacactgttttttgtattcatttgtgaatgaatgacctcttgtcagtctactcggtttcgctgtgaatgaatgatgtcttgtcagcctacttggtttcgctaagagcacagagagaagatttagtgatgctatgtaaaaacttcctttttggttcaagtgtatgtttgtgatagaaatgaagacaggctacatgatgcatatctaacataaacacaaacattaagaaaggaaatcaacctgaagagtatttatacagataacaaaatacagagagtgagttaaatgtgtaataactgtggcacaggctggaatatgagccatttaaatcacaaattaattagaaaaaaaacagtggggaaaaaattccatggatgggtctagaaagactagcattgttttaggttgagtggcagtgtttaaagggtgatatcagactaaacttgaaatatgtggctaaataactagaatactctttattttttcgtatcatgaatagcagatatagcttgatggccccatgcttggtttaacatccttgctgttcctgacatgaaatccttaatttttgacaaaggggctattcattttcattttatattgggcctagaaattatgtagatggtcctgaggaaaagtttatagcttgtctatttctctctctaacatagttgtcagcacaatgcctaggctataggaagtactcaaagcttgttaaattgaattctatccttcttattcaattctacacatggaggaaaaactcatcagggatggaggcacgcctctaaggaaggcaggtgtggctctgcagtgtgattgggtacttgcaggacgaagggtggggtgggagtggctaaccttccattcctagtgcagaggtcacagcctaaacatcaaattccttgaggtgcggtggctcactcctgtaatcacagcagtttgggacgccaaggtgggcagatcacttgaggtcaggagttggacaccagcccagccaacatagtgaaacctggtctctgcttaaaaatataaaaattagctggacgtggtgacgggagcctgtaatccaactacttgggaggctgaggcaggagaatcgcttgaaccggggaggtggagtttgcactgagcagagatcatgccattgcactccagcctccagagcgagactctgtctaaagaaaaacgaaaacaaacaaacaaacaaacaaacaaaacccatcaaattccctgaccgaacagaattctgtctgattgttctctgacttatctaccattttccctccttaaagaaactgtgaacttccttcagctagaggggcctggctcagaagcctctggtcagcatccaagaaatacttgatgtcactttggctaaaggtatgatgtgtagacaagctccagagatggtttctcatttccatatccacccacccagctttccaattttaaagccaattctgaggtagagactgtgatgaacaaacaccttgacaaaattcaacccaaagactcactttgcctagcttcaaaatccttactctgacatatactcacagccagaaattagcatgcactagagtgtgcatgagtgcaacacacacacacaccaattccatattctctgtcagaaaatcctgttggtttttcgtgaaaggatgttttcagaggctgaccccttgccttcacctccaatgctaccactctggtctaagtcactgtcaccaccacctaaattatagctgttgactcataacaatcttcctgcttctaccactgccccactacaatttcttcccaatatactatccaaattagtcttttcaaaatgtaagtcatatatggtcacctctttgttcaaagtcttctgatagtttcctatatcatttataataaaaccaaatccttacaattctctacaatagttgttcatgcatatattatgtttattacagatacatatatatagctctcatataaataaatatatatatttatgtgtatgtgtgtagagtgttttttcttacaactctatgatgtaggtattattagtgtcccaaattttataatttaggacttctatgatctcatcttttattctccccttcaccgaatctcatcctacattggccttattgatattccttgaaaattctaagcatcttacatctttagggtatttacatttgccattccctatgccctaaatatttaatcatagtttcatataaatgggttcctcatcatctatgggtactctctcaggtgttaactttatagtgaggactttcctgccatactacttaaagtagcgataccctttcaccctgtcctaatcacactctggccttcatttcagttttttttttttctccatagcacctaatctcattggtatataacatgtttcatttgcttatttaatgtcaagctctttccactatcaagtccatgaaaacaggaactttattcctctattctgtttttgtgctgtattcttagcaattttacaattttgaatgaatgaatgagcagtcaaacacatatacaactataattaaaaggatgtatgctgacacatccactgctatgcacacacaaagaaatcagtggagtagagctggaagtgctaagcctgcatagagctagttagccctccgcaggcagagccttgatgggattactgagttctagaattggactcatttgttttgtaggctgagatttgctcttgaaaacttgttctgaccaaaataaaaggctcaaaagatgaatatcgaaaccagggtgttttttacactggaatttataactagagcactcatgtttatgtaagcaattaattgtttcatcagtcaggtaaaagtaaagaaaaactgtgccaaggcaggtagcctaatgcaatatgccactaaagtaaacattatttcataggtgtcagatatggcttattcatccatcttcatgggaaggatggccttggcctggacatcagtgttatgtgaggttcaaaacacctctaggctataaggcaacagagctccttttttttttttctgtgctttcctggctgtccaaatctctaatgataagcatacttctattcaatgagaatattctgtaagattatagttaagaattgtgggagccattccgtctcttatagttaaatttgagcttcttttatgatcactgtttttttaatatgctttaagttctggggtacatgtgccatggtggtttgctgcacccatcaacccgtcatctacattaggtatttctcctaatgctatccttcccctagccccccacccccaacaggccccagtgtgtgatgttcccctccctgtgtccatggatcactggtttttttttgttttttttttttttttaaagtctcagttaaatttttggaatgtaatttattttcctggtatcctaggacttgcaagttatctggtcactttagccctcacgttttgatgataatcacatatttgtaaacacaacacacacacacacacacacacacatatatatatatataaaacatatatatacataaacacacataacatatttatcgggcatttctgagcaactaatcatgcaggactctcaaacactaacctatagccttttctatgtatctacttgtgtagaaaccaagcgtggggactgagaaggcaatagcaggagcattctgactctcactgcctttagctaggcccctccctcatcacagctcagcatagtcctgagctcttatctatatccacacacagtttctgacgctgcccagctatcaccatcccaagtctaaagaaaaaaataatgggtttgcccatctctgttgattagaaaacaaaacaaaataaaataagcccctaagctcccagaaaacatgactaaaccagcaagaagaagaaaatacaataggtatatgaggagactggtgacactagtgtctgaatgaggcttgagtacagaaaagaggctctagcagcatagtggtttagaggagatgtttctttccttcacagatgccttagcctcaataagcttgcggttgtggaagtttactttcagaacaaactcctgtggggctagaattattgatggctaaaagaagcccgggggagggaaaaatcattcagcatcctcacccttagtgacacaaaacagagggggcctggttttccatatttcctcatgatggatgatctcgttaatgaaggtggtctgacgagatcattgcttcttccatttaagccttgctcacttgccaatcctcagttttaaccttctccagagaaatacacattttttattcaggaaacatactatgttatagtttcaatactaaataatcaaagtactgaagatagcatgcataggcaagaaaaagtccttagctttatgttgctgttgtttcagaatttaaaaaagatcaccaagtcaaggacttctcagttctagcactagaggtggaatcttagcatataatcagaggtttttcaaaatttctagacataagattcaaagccctgcacttaaaatagtctcatttgaattaactctttatataaattgaaagcacattctgaactacttcagagtattgttttatttctatgttcttagttcataaatacattaggcaatgcaatttaattaaaaaaacccaagaatttcttagaattttaatcatgaaaataaatgaaggcatctttacttactcaaggtcccaaaaggtcaaagaaaccaggaaagtaaagctatatttcagcggaaaatgggatatttatgagttttctaagttgacagactcaagttttaaccttcagtgcccatcatgtaggaaagtgtggcataactggctgattctggctttctactcctttttcccattaaagatccctcctgcttaattaacattcacaagtaactctggttgtactttaggcacagtggctcccgaggtcagtcacacaataggatgtctgtgctccaagttgccagagagagagattactcttgagaatgagcctcagccctggctcaaactcacctgcaaacttcgtgagagatgaggcagaggtacactacgaaagcaacagttagaagctaaatgatgagaacacatggactcatagagggaaacaacgcatactggggcctatcagagggtggagggtgagagaaggagaggatcaggaaaaatcactaatggatgctaagcgtaatacctgagtgatgagatcatctatacaacaaacccccttgacattcatttatctatgtaacaaacctgcacatcctgtacatgtacccctgaacttaaaataaaagttgaaaacaagaaagcaacagtttgaacacttgttatggtctattctctcattctttacaattacactagaaaatagccacaggcttcctgcaaggcagccacagaatttatgacttgtgatatccaagtcattcctggataatgcaaaatctaacacaaaatctagtagaatcatttgcttacatctatttttgttctgagaatatagatttagatacataatggaagcagaataatttaaaatctggctaatttagaatcctaagcagctcttttcctatcagtggtttacaagccttgtttatatttttcctattttaaaaataaaaataaagtaagttatttgtggtaaagaatattcattaaagtatttatttcttagataataccatgaaaaacattcagtgaagtgaagggcctactttacttaacaagaatctaatttatataatttttcatactaatagcatctaagaacagtacaatatttgactcttcaggttaaacatatgtcataaattagccagaaagatttaagaaaatattggatgtttccttgtttaaattaggcatcttacagtttttagaatcctgcatagaacttaagaaattacaaatgctaaagcaaacccaaacaggcaggaattaatcttcatcgaatttgggtgtttctttctaaaagtcctttatacttaaatgtcttaagacatacatagattttattttactaattttaattatatagacaataaatgaatattcttactgattactttttctgactgtctaatctttctgatctatcctggatggccataacacttatctctctgaactttgggcttttaatataggaaagaaaagcaataatccatttttcatggtatctcatatgataaacaaataaaatgcttaaaaatgagcaggtgaagcaatttatcttgaaccaacaagcatcgaagcaataatgagactgcccgcagcctacctgacttctgagtcaggatttataagccttgttactgagacacaaacctgggcctttcaatgctataacctttcttgaagctcctccctaccacctttagccataaggaaacatggaatgggtcagatccctggatgcaagccaggtctggaaccataggcagtaaggagagaagaaaatgtgggctctgcaactggctccgagggagcaggagaggatcaaccccatactctgaatctaagagaagactggtgtccatactctgaatgggaagaatgatgggattacccatagggcttgttttagggagaaacctgttctccaaactcttggccttgagatacctggtccttattccttggactttggcaatgtctgaccctcacattcaagttctgaggaagggccactgccttcatactgtggatctgtagcaaattccccctgaaaacccagagctgtatcttaattggttaaaaaaaattatattatctcaacgactgttcttctctgagtagccaagctcagcttggttcaagctacaagcagctgagctgctttttgtctagtcattgttcttttatttcagtggatcaaatacgttctttccaaacctaggatcttgtcttcctaggctatatattttgtcccaggaagtcttaatctggggtccacagaacactagggggctggtgaagtttatagaaaaaaaatctgtatttttacttacatgtaactgaaatttagcattttcttctactttgaatgcaaaggacaaactagaatgacatcatcagtacctattgcatagttataaagagaaaccacagatattttcatactacaccataggtattgcagatctttttgtttttgtttttgtttgagatggagtttcgctcttattgcccaggctggagtgcagtggcatgatttcggctcactgcaacctccccttcctgcattcaagcaattctcctgccttggcctcctgagtagctggggattacaggcacctgccaccatgccagtctaatttttgtatttttagtagagatggggtttcgccatgttggccaggctggtcttgaactcctgacctcagatgatctgcccgccttggcctcctgaagtgctgggattataggtgtgagccaccacgcctggcccattgcagatatttttaattcacatttatctgcatcactacttggatcttaaggtagctgtagacccaatcctagatctaatgctttcataaagaagcaaatataataaatactataccacaaatgtaatgtttgatgtctgataatgatatttcagtgtaattaaacttagcactcctatgtatattatttgatgcaataaaaacatatttttttagcacttacagtctgccaaactggcctgtgacacaaaaaaagtttaggaattcctggttttgtctgtgttagccaatggttagaatatatgctcagaaagataccattggttaatagctaaaagaaaatggagtagaaattcagtggcctggaataataacaatttgggcagtcattaagtcaggtgaagacttctggaatcatgggagaaaagcaagggagacattcttacttgccacaagtgtttttttttttttttttttttatcacaaacataagaaaatataataaataacaaagtcaggttatagaagagagaaacgctcttagtaaacttggaatatggaatccccaaaggcacttgacttgggagacaggagccatactgctaagtgaaaaagacgaagaacctctagggcctgaacatacaggaaattgtaggaacagaaattcctagatctggtggggcaaggggagccataggagaaagaaatggtagaaatggatggagacggaggcagaggtgggcagatcatgaggtcaagagatcgagaccatcctggcaaacatggtgaaatcccgtctctactaaaaataaaaaaattagctgggcatggtggcatgcgcctgtagtcccagctgctcgggaggctgaggcaggagaatcgtttgaacccaggaggcgaaggttgcagtgagctgagatagtgccattgcactccagtctggcaacagagtgagactccgtctcaaaaaaaaaaaaaaaagaaagaaagaaaagaaaaagaaaaaagaaaaaataaatggatgtagaacaagccagaaggaggaactgggctggggcaatgagattatggtgatgtaagggacttttatagaattaacaatgctggaatttgtggaactctgcttctattattcccccaatcattacttctgtcacattgatagttaaataatttctgtgaatttattccttgattctaaaatatgaggataatgacaatggtattataagggcagattaagtgatatagcatgagcaatattcttcaggcacatggatcgaattgaatacactgtaaatcccaacttccagtttcagctctaccaagtaaagagctagcaagtcatcaaaatggggacatacagaaaaaaaaaaggacactagaggaataatataccctgactcctagcctgattaatatatcgattcacttttttctctgtttgatgacaaattctggctttaaataattttaggattttaggcttctcagctcccttcccagtgagaagtataagcaggacagacaggcaagcaagaagagagccccaggcaatactcacaaagtagccaatgtcccctgtggtcatagagaaatgaaaagagagaggattctctggaagcactggatgtaatcttttctgtctgtcctctctagggaatcaccccaaggtactgtactttgggattaaggctttagtcccactgtggactacttgctattctgttcagtttctagaaggaactatgtacggtttttgtctccctagagaaactaaggtacagaagttttgtttacaatgcactccttaagagagctagaactgggtgagattctgttttaacagctttattttcttttccttggccctgtttttgtcactgtcaccacctttaaggcaaatgttaaatgcgctttggctgaaactttttttcctattttgagatttgctcctttatatgaggctttcttggaaaaggagaatgggagagatggatatcattttggaagatgatgaagagggtaaaaaaggggacaaatggaaatttgtgttgcagatagatgaggagccaacaaaaaagagcctcaggatccagcacacattatcacaaacttagtgtccatccatcactgctgaccctctccggacctgactccacccctgagggacacaggtcagccttgaccaatgacttttaagtaccatggagaacagggggccagaacttcggcagtaaagaataaaaggccagacagagaggcagcagcacatatctgcttccgacacagctgcaatcactagcaagctctcaggcctggcatcatggtgcattttactgctgaggagaaggctgccgtcactagcctgtggagcaagatgaatgtggaagaggctggaggtgaagccttgggcaggtaagcattggttctcaatgcatgggaatgaagggtgaatattaccctagcaagttgattgggaaagtcctcaagattttttgcatctctaattttgtatctgatatggtgtcatttcatagactcctcgttgtttacccctggacccagagattttttgacagctttggaaacctgtcgtctccctctgccatcctgggcaaccccaaggtcaaggcccatggcaagaaggtgctgacttcctttggagatgctattaaaaacatggacaacctcaagcccgcctttgctaagctgagtgagctgcactgtgacaagctgcatgtggatcctgagaacttcaaggtgagttcaggtgctggtgatgtgattttttggctttatattttgacattaattgaagctcataatcttattggaaagaccaacaaagatctcagaaatcatgggtcgagcttgatgttagaacagcagacttctagtgagcataaccaaaacttacatgattcagaactagtgacagtaaaggactactaacagcctgaattggcttaacttttcaggaaatcttgccagaacttgatgtgtttatcccagagaattgtattatagaattgtagacttgtgaaagaagaatgaaatttggcttttggtagatgaaagtccatttcaaggaaatagaaatgccttattttatgtgggtcatgataattgaggtttagaaagagatttttgcaaaaaaaataaaagatttgctcaaagaaaaataagacacattttctaaaatatgttaaatttcccatcagtattgtgaccaagtgaaggcttgtttccgaatttgttggggattttaaactcccgctgagaactcttgcagcactcacattctacatttacaaaaattagacaattgcttaaagaaaaacagggagagagggaacccaataatactggtaaaatggggaagggggtgagggtgtaggtaggtagaatgttgaatgtagggctcatagaataaaattgaacctaagctcatctgaattttttgggtgggcacaaaccttggaacagtttgaggtcagggttgtctaggaatgtaggtataaagccgtttttgtttgtttgtttgttttttcatcaagttgttttcggaaacttctactcaacatgcctgtgtgttattttgtcttttgcctaacagctcctgggtaacgtgatggtgattattctggctactcactttggcaaggagttcacccctgaagtgcaggctgcctggcagaagctggtgtctgctgtcgccattgccctggcccataagtaccactgagttctcttccagtttgcaggtgttcctgtgaccctgacaccctccttctgcacatggggactgggcttggccttgagagaaagccttctgtttaataaagtacattttcttcagtaatcaaaaattgcaattttatcttctccatcttttactcttgtgttaaaaggaaaaagtgttcatgggctgagggatggagagaaacataggaagaaccaagagcttccttaagaaatgtatgggggcttgtaaaattaatgtggatgttatgggagaattccaggattccaaggaggatgatatgatggagaaaaatctttatcggggtgggaaaatggttaattaagtggacagagactcctaggcagtttttactgcaccggggaaagaaggagctgttagtggtacctgagaaagcagatttgtggtacatgtcacttttcattaaaaacaaaaacaaaacaaaacaaaacttcatagatatccaagatataggctagaattactattttaatttactcttatttacattttgaagtagctagcttgtcacatgttttatgaaattgatttggagataagatgagtgtgtatcaacaatagcctgctctttccatgaaggattccattatttcatgggttagctgaagctaagacacatgatatcattgtgcattatcttctgatagaatgtaacatgcactaaaataaagttagagttaggacctgagtgggaaagtttttggagagtgtgatgaagactttccgtgggagatagaatactaataaaggcttaaattctaaaaccagcaagctagggcttcgtgacttgcatgaaactggctctctggaagtagaagggagagtaagacatacgtagaggactaggaaagaccagatagtacagggcctggctacaaaaatacaagcttttactatgctattgcaatactaaacgataagcattaggatgttaagtgactcaggaaataagattttgggaaaaagtaatctgcttatgtgcacaaaatggattcaagtttgcagataaaataaaatatggatgatgattcaaggggacagatacaatggttcaaacccaagaggagcagtgagtctgtggaatttgaaggatggacaaaggtggggtgagaaagacatagtattcgactgactgtgggagatgagaaggaagaaggaggtgataaatgactgaaagctcccagactggtgaagataacaggaggaaaccatgcactgacctggtgactctcatgtgtgaagggtagagggatattaacagatttactttttaggaagtgctagattggtcagggagttttgaccttcaggtcttgtgtctttcatatcaaggaacctttgcattttccaagttagagtgccatattttggcaaatataactttattagtaattttatagtgctctcacattgatcagactttttcctgtgaattacttttgaatttggctgtatatatccagaatatgggagagagacaaataattattgtagttgcaggctatcaacaatactggtctctctgagccttataacctttcaatatgcccataaacagagtaaacagggattattcatggcactaaatattttcacctagtcagtcaacaaatgggagcaatgtgcattttttgatacatatttttatatatttatggggtacatgtgatacttacatgcctagaacatgtgatgattaagtctagatatttaggatatccattgctttgagcatttatcatttctatgtattgagaaaatttcaaatcctcatttctagccattttgaaatatataataaatagtaattaactatagtcaccctactcaaatatcaaacattatggcttaatccttctatccaactgtgtttgtacctattaaccaacatctcttaaatcccctcccatacacactcacactttttccagcctctgataactatcattctactctctaccaccatgagacccacttttttagctcccacagatgaataaaaacatgtgatatttgactttctgtatctggcttattttattatctatctctttggcataccaagagtttgtttttgttctgcttcagggctttcaattaacataatgacctctggttccatccatgttgctacaaatgacaagatttcattctttttcatggcaaaatagtactgtgcaaaaatacaattttttaatccgttcatctgttgatagacacttaggttgatcccaaaccttaactattgtgaatagtgcttcaataaacatgagtgtaatgtgtccattggatatactgatttcctttcttttggataaataaccactagtgagattgctggattgtatgatagttctgtttttagtttactgagaaatcttcatactgttttccataatggttgtactattttacattcccaccaacagtgtgtaagaaagagttcccttttctccatatcctcacaaggatctgttattttttgtcttttttgttaatagccgttttaactagagtaagtagatatctcattgtagttttgatttgcatttccctgatcattagtgatgttgagaattttttcatatgtttgttggtcatttgtatatctttttctgagaattgtctgttcatgtccttagcctactttttattgggattgtttgttattttcttgataatctatttgtgttcattttagagcctggatattattcttttgtcagatgtatagattgtgaagattttctcccactctgtgggttgtctgtttattctgcagactcttccttttgccatgcaaaagctctttagtttaatttagtcccagatattttctttgtttttatgtatttgcatttgtgttcttggtcatgaaatcctttcctaagccaatgtgtagaagggtttttccgatgttattttctagaattgttacagtttcagggcttagatttaagtccttgatccatcttgagttgatttttgtataaggtgagagatgaagatccagtttcattctcctacatgtagcttgccagctatccccgcaccatttgttgaatagggtgccctttccccactttatgtttttgtttgctttgtcaaagatcagttggatgtaagtatttgagtttatttctgggttctctattctgttccattggtcgatgtgcctatttgtacaccagcatcatgctgttttggtgactatggccttattgtatagtttgaaatgaggtaatgtaatgccttcagatttgttcttttttttagacttgcttgtttattgggctcttttttggttccataagaattttaggattgttttttctagttctgtgaagactaatggtggtattttgatgggaattgcaatgaatttgtaggttgcttctggcattatggccattttcacaatattgattctacccatctatgagaatggcatgtgtttccatttgtttgtgtcttatatgattactttcagccgtgttttgtagttttccttgtagatgtctttcacctccttggttaggtatatattcctaagtttttgttttgttttgttttgttttttgcagctattgtaaaaggggttgagttcttgattttattctcagcttggtcattgctggtatgtaagaaagcaactcattggtgtacgttaattttgtatccagaaactttgctgaattattttatcagttctagggggttttggaggagtctttagagttttctacatacacaatcatatcatcagcaaacagtgacagtttgactttctctttaacaatttggatgtgctttacttgtttctcttgtctgattgctcttgctaggacttccagtaatatgttaaagagaagtggtgagagtgggtatccttgtctcattccagttttcagacagaatgcttttaactttttcccattcaatataatgttggctgtgtgtttaccatagctggcttttattacattgaggtatgtcctttgtaaaccgattttgctgagttttagtcataaagtgatgttgaattttgttgaatgcagtttctgtggctattgagataatcacatgatttttgtttccaattctctttatgttgtgtatcacacttattgacttgcgtatgttaaaccatccgtgcatccctcgcatgaaacccacttgatcatgggttttgatatgctgtcggatgctattagctagtattttgtcaaggatgttggcatctatgttcatcagggatattgatctgtagtgttttttttttttggttatgttctttcccagttttggtattaaggtgatactggcttcatagaatgatttagggaggattctctctttctctatcttgtagaatactgtcaataggattggtatcaattcttctttgaatgtctggtagaattcagctgtgaatctatctggtcctggacttttttgttgttggtaaatttttattatcatttcagtcttgctgcttattactggtctgttcagggtatctaattcttcctgacttaagctagagccctgtatctttccaggaattcgaacgtctcctttaggttttctagtttatgcatgtaaaggtgttcatagtagccttgaataatcttttgtatttctgtggtatcagtaatagtatctcctgttttgtttctaattgagtttatttgcacttctctcctcttttcttggttaatcttgctaatggtctatcagttttatttatcttttcaaagaaccagctttttatttcatttagcttttgtatttttttgcagttgttttaatttcatttagttctcctcttatcttagttattccctttcttttgctgggttttggttctgtttgtttttgtttctctagtttcttgtggtgtgaccttatattgtctgtctgtcctctttcagactctttgacatcgacatttagggctgtgaactttccttttagcaccatctttgctgtatcctagaggttttgataggttgtgtcactattgtcggtcagttcaagtaattttgttgttcttattatactttaagttctgggatacatgtgcagaatgtgcaggtttgttacataggtatagatgtgccatggtggtttgctgcacccatcaacctgtcatctacattaggtatttcttttaatgttatccctctcctaaccccctcaccccccgacaggccctggtgtgtgatgttcccctccctgtgtccatgtgttctcattgttcaactcccacttatgagtgagaacgtgtggtgtttggtttctctgttcctgtgttagtttgctcagaatgatggtttccaccttcatccatgtccctgcaaagacatgaactcatcatttttatggctgcatagtattccatggtgtatatgtgccacattttctttatccattatatcgctgatggccatttgggttggttccaagtctttgctattgtgaatagtgccacaataaacatacgtgtgcacgtgtctttatagtagaatgatttctaattctttgggtatatacccagtaatgggattgctgggtcaaacagtatttctggttctagatccttgaggaatcgccacactgtcttccacaatggttgaactaatttacacacccatcaacagtgtaaaatttttcctattcttccacatcctctccagcaccttttgtttcctgactttttaataattgccattctaactggcatgagatggtatctcattgtggttttgatttgcatttctctaatgaccagtgatgatgagcttcttttcatgtgtttcttggccacataaatgacttctttagagaagcatctgttcatatcctttgtccactttttgatggggtcgttaggttttttcttgtaaatttgttgaagttctttgtagattttggatgttagccctttgtcagatggatagattgcaaaaattttctcccattctgtaggttgcctgttcactctgatgatagtcttttgctgtgcagaagctctttagtttaattagatcccatatgtcaattttggcctttgttgtcattgcttttgatgttttagtcgtgaatttttgcccatgcctatgtcctgaatggtattgcctaggttatcttctaggatttttatggttttaggttgcacatttaagtctttaatccaccttgagttaatttttgtataaggtgtaaggaaggggtacagtttcagttttatgcatattgctagccagtttttccagcaccatttattaaatagggaattctttctccattgcttttgtgatgtttgtcaaagatcagatggtcgtagatgtgtggcattatttctgaggcttctgttctgttccactggtctatatatctgttttggtaccagtaccatgctgtttttgttactgtagccttgtagtatagtttgaagtcaggtagcatcatgcctccagctttgttctttttgtttaggattgtcttggctatatgggctcttttttgattccatatgacatttaaagtagttttttctaattctttgaaaaaagtcagtggtagcttgatggggatagcattgaatctataaattactttgggcagtatggccattttaaagatattgattctttctatctatgagcatggaatgtttttccatttgtttgtgtcctctcttatttccttgagcagtgagtggtttgtagctctccttgaagaggttcttcacatcccttagaagttgtatttctaggtattttattttattctctttgcagcaattgtgaatgggagttcacccatgatttggctctctgcttgtctattattggtgtataggaacgcttgtgatttctgcacactgattttgtatcttgagactttgctgaagctgtttatcagcttaagattttgggctgagatgacagggtcttctaaatatacaatcatgtcatctgcaaacagagacaatttgacttcctctcttcctatttgaatatgctttatttctttctcttgcctgattgtcctggcgagaacttccaatactatgttgagtaagagtggcgagagggcatccttgtcttgtgccggttttcaaagcaaatgatttttaaatttccatcttgatttcattgttgacccaatgatcattcaggagcaggttatttaatttccctgtatttgcatggttttgaaggttccttttgtagttgatttccaattttattctactgtggtctgagagagtgcttgatataatttcaatttttaaaaatttattgaggcttgttttgtggcatatcatatggcctatcttggagaaagttccatgtgctgatgaatagaatgtgtattctgcagttgttgggtagaatgtcctgtaaatatctgttaagtccatttgttctttaaatccattgtttctttgtagactgtcttgatgacctgcctagtgcagtcagtggagtattgaagtcccccactattattatgttgctgtctagtctagtagtaattgttttataaatttgggatctccagtattagatgcatatatattaagaattgtaatattctcccattggacaagggcttttatcattatatgatgtccctctttgtcttttttaactgctgtttctttaaagtttgttttgtctgacataagaatagctgctttggctcgcttttggtgtccatttgtgtggaatgtcattttccacccctttaccttaagtttatgtgagtccttatgtgttaggtgagtctcctgaaggcggcagataactggttggtgaattcttattcattctgcaattctgtatcttttaagtggagcatttagtccatttacattcaacatcagtattgaggtgtgaggtactattccattcttcgtggtatttgttgcctgtgtatctttttatctgtatttttgttgtatatgtcctatgggatttatgctttaaagaggttctgttttgatgtgcttccagggtttatttcaagatttagagctccttttatcagttcttgtagtgttggcttggtagtgccgaattctctcagcatttgtttttctgaaaaacactgtgtattttcttcatttgtgaagcttagtttcactggatataaaattcttggctgataattgttttgtttaagaaggctgaagatagggccatattcacttctagcttttacggtttctgctgagaaatctgctgttaatctgataggttttctttcataggttacctggtagtttcacctcacagctcttaagattctctttgtctttagataactttggatactctgatgacaatgtacctaggcaatgatatttttgcaatgaatttcccaggtgtttattgagcttcttgtatttggatatctaggtctctagcaaggtgggggaagttttccttgattatttccctggataagttttccaaacttttagatttctcttctttctcaggaatgctgattattcttaggtttgattgtttaacataatcccagatttcttggaggctttgttcatattttcttattcttttttctttgtctttgttggattgggttaattcaaaaactttgtcttcaagctctgaatttcttctgcttggattctattgctgagactttctagagcattttgcatttctataagtgcatccattcatccattgtttcctgaagttttgaatgttttttatttatgctatctctttaactgaagatttctcccctcatttcttgtatcatatttttggtttttttaaaattggacttcaccttcctcggatgcctccttgattagcttaataactgaccttctgaattatttttcaggtaaatcagggatttcttcttggtttggatgcattgctggtgagctagtatgattttttggggggtgttaaagaaccttgtttttcatattaccagagttagttttctggttccttctcacttgggtaggctctgtcagagggaaagtctaggcctcaaggctgagacttttgtcccatgaggtgttcccttgatgtagcacagtcccccttttcctaggcgtggggcttcctgagagccgaactgtagtgattgttatctctcttctggatctagccacccatcaggtctaccagactccaggctggtactggggtttgtctgcacagagtcttgtgacgtgaaccatctgtgggtctctcagccatagatacaaccacctgctccaatggaggtggcagaggatgaaatggactctgtgagggtccttacttttggttgttcaatgcactatttttgtgctggttggcctcctgccaggaggtggcactttctagaaagcatcagcagaggcagtcaggtggtggtggctgggggggctggggcaccctagaactcccaagaatatatgccctttgtcttcagctaccagggtgagtaaggaaggaccatcaggtgggggcaggactagtcgtgtctgagctcagagtctccttgggcaggtctttctgtggctactgtgggaggatgggggtgtagtttccaggtcaatggatttatgttcctaggacaattatggctgcctctgctgtgtcatgcaggtcatcaggaaagtgggggaaagcaagcagtcacgtgacttgcccagctcccatgcaactcaaaaggttggtctcacttccagcgtgcaccctcccccgcaacagcaccgaatctgtttccatgcagtcagtgagcaaggctgagaacttgccccaggctaccagctgcgaaaccaagtagggctgtcctacttccctgccagtggagtctgcacaccaaattcatgtccccccaccaacccccccactgcccagcccctagatctggccaggtggagattttctttttcctgtcatcttttcccagttcctctggcagccctcccaaatgacccctgtgaggcaaggcagaaatggcttcctaggggacccagagagcccacagggcttttcccgctgcttcctctacccctgtattttgcttggccctctaaattgactcagctccaggtaaggtcagaatcttctcctgtggtctagatcttcaggttccccagtgaggatgtgtgtttgggggtagacggtcccccttttccacttccacagtttgggcactcacaatatttggggtgtttcccgggtcctgcaggagcaatctgcttctttcagagggtgtgtgcgttctctcagctttcttgatttatttctgcaggtggttctgcaaaaaaaattcctgatgggagacttcacatgctgctctgtgcatccgagtgggagctgcaatgtacttctgctgcctcccatctgccatcaccctctaatttgtcggtaatatgcatttttaatcaatctttttttctctctctctctttttcttctcccccaaaactatactgccctttgatatcaaggaatcaaggacgtgatgttgaggggtgggcagtggatacactctttaccccttagggagctatatctagatttagatattgccaattcaagataacttaattgaaagcaaattcataatgaatacacacacacacacacacatctgcatgacaagatttttaatagttgaaagaataactaataattgtccacaggcaataagggctttttaagcaaaacagttgtgataaacaggtcattcttagaatagtaatccagccaatagtacaggttgcttagagattatgtcattaccagagttaaaattctataatggcttctcactccctaccactgaggacaagtttatgtccttaggtttatgcttccctgaaacaataccacctgctattctccactttacatatcaacggcactggttctttatctaactctctggcacagcaggagtttgttttcttctgcttcagagctttgaatttactatttcagcttctaaactttatttggcaatgccttcccatggcagattccttctgtcattttgcctctgttcgaatactttctccttaatttcattcttagttaataatatctgaaattattttgttgtttaacttaattattaattttatgtatgttctacctagattataatcttcagaggaaagttttattctctgacttatttaacttaaatgcccactactttaaaaattatgacatttatttaacagatatttgctgaacaaatgtttgaaaatacatgggaaagaatgcttgaaaacacttgaaattgcttgtgtaaagaaacagttttatcagttaggatttaatcaatgtcagaagcaatgatataggaaaaatcgaggaataagacagttatggataaggagaaatcaacaaactcttaaaagatattgcctcaaaagcataagaggaaataagggtttatacatgacttttagaacactgccttggtttttggataaatggggaagttgtttgaaaacaggagggatcctagatattccttagtctgaggaggagcaattaagattcacttgtttagaggctgggagtggtggctcacgcctgtaatcccagaattttgggaggccaaggcaggcagatcacctgaggtcaagagttcaagaccaacctggccaacatggtgaaatcccatctctacaaaaatacaaaaattagacaggcatgatggcaagtgcctgtaatcccagctacttgggaggctgaggaaggagaattgcttgaacctggaaggcaggagttgcagtgagccgagatcataccactgcactccagcctgggtgacagaacaagactctgtctcaaaaaaaaaaaagagagattcaaaagattcacttgtttaggccttagcgggcttagacaccagtctctgacacattcttaaaggtcaggctctacaaatggaacccaaccagactctcagatatggccaaagatctatacacacccatctcacagatcccctatcttaaagagaccctaatttgggttcacctcagtctctataatctgtaccagcataccaataaaaatctttctcacccatccttagattgagagaagtcacttattattatgtgagtaactggaagatactgataagttgacaaatctttttctttcctttcttattcaacttttattttaacttccaaagaacaagtgcaatatgtgcagctttgttgcgcaggtcaacatgtatctttctggtcttttagccgcctaacactttgagcagatataagccttacacaggattatgaagtctgaaaggattccaccaatattattataattcctatcaacctgataggttaggggaaggtagagctctcctccaataagccagatttccagagtttctgacgtcataatctaccaaggtcatggatcgagttcagagaaaaaacaaaagcaaaaccaaacctaccaaaaaataaaaatcccaaagaaaaaataaagaaaaaaacagcatgaatacttcctgccatgttaagtggccaatatgtcagaaacagcactgagttacagataaagatgtctaaactacagtgacatcccagctgtcacagtgtgtggactattagtcaataaaacagtccctgcctcttaagagttgttttccatgcaaatacatgtcttatgtcttagaataagattccctaagaagtgaacctagcatttatacaagataattaattctaatccatagtatctggtaaagagcattctaccatcatctttaccgagcatagaagagctacaccaaaaccctgggtcatcagccagcacatacacttatccagtgataaatacacatcatcgggtgcctacatacatacctgaatataaaaaaaatacttttgctgagatgaaacaggcgtgatttatttcaaataggtacggataagtagatattgaagtaaggattcagtcttatattatattacataacattaatctattcctgcactgaaactgttgctttataggatttttcactacactaatgagaacttaagagataatggcctaaaaccacagagagtatattcaaagataagtatagcacttcttatttggaaaccaatgcttactaaatgagactaagacgtgtcccatcaaaaatcctggacctatgcctaaaacacatttcacaatccctgaacttttcaaaaattggtacatgctttaactttaaactacaggcctcactggagctacagacaagaaggtgaaaaacggctgacaaaagaagtcctggtatcttctatggtgggagaagaaaactagctaaagggaagaataaattagagaaaaattggaatgactgaatcggaacaaggcaaaggctataaaaaaaattaagcagcagtatcctcttgggggccccttccccacactatctcaatgcaaatatctgtctgaaacggtccctggctaaactccacccatgggttggccagccttgccttgaccaatagccttgacaaggcaaacttgaccaatagtcttagagtatccagtgaggccaggggccggcggctggctagggatgaagaataaaaggaagcacccttcagcagttccacacactcgcttctggaacgtctgaggttatcaataagctcctagtccagacgccatgggtcatttcacagaggaggacaaggctactatcacaagcctgtggggcaaggtgaatgtggaagatgctggaggagaaaccctgggaaggtaggctctggtgaccaggacaagggagggaaggaaggaccctgtgcctggcaaaagtccaggtcgcttctcaggatttgtggcaccttctgactgtcaaactgttcttgtcaatctcacaggctcctggttgtctacccatggacccagaggttctttgacagctttggcaacctgtcctctgcctctgccatcatgggcaaccccaaagtcaaggcacatggcaagaaggtgctgacttccttgggagatgccataaagcacctggatgatctcaagggcacctttgcccagctgagtgaactgcactgtgacaagctgcatgtggatcctgagaacttcaaggtgagtccaggagatgtttcagcactgttgcctttagtctcgaggcaacttagacaactgagtattgatctgagcacagcagggtgtgagctgtttgaagatactggggttgggagtgaagaaactgcagaggactaactgggctgagacccagtggcaatgttttagggcctaaggagtgcctctgaaaatctagatggacaactttgactttgagaaaagagaggtggaaatgaggaaaatgacttttctttattagatttcggtagaaagaactttcacctttcccctatttttgttattcgttttaaaacatctatctggaggcaggacaagtatggtcattaaaaagatgcaggcagaaggcatatattggctcagtcaaagtggggaactttggtggccaaacatacattgctaaggctattcctatatcagctggacacatataaaatgctgctaatgcttcattacaaacttatatcctttaattccagatgggggcaaagtatgtccaggggtgaggaacaattgaaacatttgggctggagtagattttgaaagtcagctctgtgtgtgtgtgtgtgtgtgtgcgcgcgtgtgtttgtgtgtgtgtgagagcgtgtgtttcttttaacgttttcagcctacagcatacagggttcatggtggcaagaagataacaagatttaaattatggccagtgactagtgctgcaagaagaacaactacctgcatttaatgggaaagcaaaatctcaggctttgagggaagttaacataggcttgattctgggtggaagcttggtgtgtagttatctggaggccaggctggagctctcagctcactatgggttcatctttattgtctcctttcatctcaacagctcctgggaaatgtgctggtgaccgttttggcaatccatttcggcaaagaattcacccctgaggtgcaggcttcctggcagaagatggtgactggagtggccagtgccctgtcctccagataccactgagctcactgcccatgatgcagagctttcaaggataggctttattctgcaagcaatcaaataataaatctattctgctaagagatcacacatggttgtcttcagttctttttttatgtctttttaaatatatgagccacaaagggttttatgttgagggatgtgtttatgtgtatttatacatggctatgtgtgtttgtgtcatgtgcacactccacacttttttgtttacgttagatgtgggttttgatgagcaaataaaagaactaggcaataaagaaacttgtacatgggagttctgcaagtgggagtaaaaggtgcaggagaaatctggttggaagaaagacctctataggacaggactcctcagaaacagatgttttggaagagatggggaaaggttcagtgaagggggctgaacccccttccctggattgcagcacagcagcgaggaaggggctcaacgaagaaaaagtgttccaagctttaggaagtcaaggtttaggcagggatagccattctattttattaggggcaatactatttccaacggcatctggcttttctcagcccttgtgaggctctacagggaggttgaggtgttagagatcagagcaggaaacaggtttttctttccacggtaactacaatgaagtgatccttactttactaaggaacttttcattttaagtgttgacgcatgcctaaagaggtgaaattaatcccatacccttaagtctacagactggtcacagcatttcaaggaggagacctcattgtaagcttctagggaggtggggacttaggtgaaggaaatgagccagcagaagctcacaagtcagcatcagcgtgtcatgtctcagcagcagaacagcacggtcagatgaaaatatagtgtgaagaatttgtataacattaattgagaaggcagattcactggagttcttatataattgaaagttaatgcacgttaataagcaagagtttagtttaatgtgatggtgttatgaacttaacgcttgtgtctccagaaaattcacatgctgaatccccaactcccaattggctccatttgtgggggaggctttggaaaagtaatcaggtttagaggagctcatgagagcagatccccatcatagaattattttcctcatcagaagcagagagattagccatttctcttccttctggtgaggacacagtgggaagtcagccacctgcaacccaggaagagagccctgaccaggaaccagcagaaaagtgagaaaaaatcctgttgttgaagtcacccagtctatgctattttgttatagcaccttgcactaagtaaggcagatgaagaaagagaaaaaaataagcttcggtgttcagtggattagaaaccatgtttatctcaggtttacaaatctccacttgtcctctgtgtttcagaataaaataccaactctactactctcatctgtaagatgcaaatagtaagcctgagcccttctgtctaactttgaattctattttttcttcaacgtactttaggcttgtaatgtgtttatatacagtgaaatgtcaagttctttctttatatttctttctttcttttttttcctcagcctcagagttttccacatgcccttcctactttcaggaacttctttctccaaacgtcttctgcctggctccatcaaatcataaaggacccacttcaaatgccatcactcactaccatttcacaattcgcactttctttctttgtcctttttttttttagtaaaacaagtttataaaaaattgaaggaataaatgaatggctacttcataggcagagtagacgcaagggctactggttgccgatttttattgttatttttcaatagtatgctaaacaaggggtagattatttatgctgcccatttttagaccataaaagataacttcctgatgttgccatggcatttttttccttttaattttatttcatttcattttaatttcgaaggtacatgtgcaggatgtgcaggcttgttacatgggtaaatgtgtgtctttctggccttttagccatctgtatcaatgagcagatataagctttacacaggatcatgaaggatgaaagaatttcaccaatattataataatttcaatcaacctgatagcttaggggataaactaatttgaagatacagcttgcctccgataagccagaattccagagcttctggcattataatctagcaaggttagagatcatggatcactttcagagaaaaacaaaaacaaactaaccaaaagcaaaacagaaccaaaaaaccaccataaatacttcctaccctgttaatggtccaatatgtcagaaacagcactgtgttagaaataaagctgtctaaagtacactaatattcgagttataatagtgtgtggactattagtcaataaaaacaacccttgcctctttagagttgttttccatgtacacgcacatcttatgtcttagagtaagattccctgagaagtgaacctagcatttatacaagataattaattctaatccacagtacctgccaaagaacattctaccatcatctttactgagcatagaagagctacgccaaaaccctgggtcatcagccagcacacacacttatccagtggtaaatacacatcatctggtgtatacatacatacctgaatatggaatcaaatatttttctaagatgaaacagtcatgatttatttcaaataggtacggataagtagatattgaggtaagcattaggtcttatattatgtaacactaatctattactgcgctgaaactgtggctttatagaaattgttttcactgcactattgagaaattaagagataatggcaaaagtcacaaagagtatattcaaaaagaagtatagcactttttccttagaaaccactgctaactgaaagagactaagatttgtcccgtcaaaaatcctggacctatgcctaaaacacatttcacaatccctgaacttttcaaaaattggtacatgctttagctttaaactacaggcctcactggagctagagacaagaaggtaaaaaacggctgacaaaagaagtcctggtatcctctatgatgggagaaggaaactagctaaagggaagaataaattagagaaaaactggaatgactgaatcggaacaaggcaaaggctataaaaaaaattagcagtatcctcttgggggccccttccccacactatctcaatgcaaatatctgtctgaaacggtccctggctaaactccacccatgggttggccagccttgccttgaccaatagccttgacaaggcaaacttgaccaatagtcttagagtatccagtgaggccaggggccggcggctggctagggatgaagaataaaaggaagcacccttcagcagttccacacactcgcttctggaacgtctgaggttatcaataagctcctagtccagacgccatgggtcatttcacagaggaggacaaggctactatcacaagcctgtggggcaaggtgaatgtggaagatgctggaggagaaaccctgggaaggtaggctctggtgaccaggacaagggagggaaggaaggaccctgtgcctggcaaaagtccaggtcgcttctcaggatttgtggcaccttctgactgtcaaactgttcttgtcaatctcacaggctcctggttgtctacccatggacccagaggttctttgacagctttggcaacctgtcctctgcctctgccatcatgggcaaccccaaagtcaaggcacatggcaagaaggtgctgacttccttgggagatgccacaaagcacctggatgatctcaagggcacctttgcccagctgagtgaactgcactgtgacaagctgcatgtggatcctgagaacttcaaggtgagtccaggagatgtttcagccctgttgcctttagtctcgaggcaacttagacaacggagtattgatctgagcacagcagggtgtgagctgtttgaagatactggggttgggggtgaagaaactgcagaggactaactgggctgagacccagtggtaatgttttagggcctaaggagtgcctctaaaaatctagatggacaattttgactttgagaaaagagaggtggaaatgaggaaaatgacttttctttattagattccagtagaaagaactttcatctttccctcatttttgttgttttaaaacatctatctggaggcaggacaagtatggtcgttaaaaagatgcaggcagaaggcatatattggctcagtcaaagtggggaactttggtggccaaacatacattgctaaggctattcctatatcagctggacacatataaaatgctgctaatgcttcattacaaacttatatcctttaattccagatgggggcaaagtatgtccaggggtgaggaacaattgaaacatttgggctggagtagattttgaaagtcagctctgtgtgtgtgtgtgtgtgtgcgcgcgcgcgtgtgtgtgtgtgtgtcagcgtgtgtttcttttaacgtcttcagcctacaacatacagggttcatggtggcaagaagatagcaagatttaaattatggccagtgactagtgcttgaaggggaacaactacctgcatttaatgggaaggcaaaatctcaggctttgagggaagttaacataggcttgattctgggtggaagcttggtgtgtagttatctggaggccaggctggagctctcagctcactatgggttcatctttattgtctcctttcatctcaacagctcctgggaaatgtgctggtgaccgttttggcaatccatttcggcaaagaattcacccctgaggtgcaggcttcctggcagaagatggtgactgcagtggccagtgccctgtcctccagataccactgagctcactgcccatgattcagagctttcaaggataggctttattctgcaagcaatacaaataataaatctattctgctgagagatcacacatgattttcttcagctcttttttttacatctttttaaatatatgagccacaaagggtttatattgagggaagtgtgtatgtgtatttctgcatgcctgtttgtgtttgtggtgtgtgcatgctcctcatttatttttatatgagatgtgcattttgatgagcaaataaaagcagtaaagacacttgtacacgggagttctgcaagtgggagtaaatggtgtaggagaaatccggtgggaagaaagacctctataggacaggacttctcagaaacagatgttttggaagagatgggaaaaggttcagtgaagacctgggggctggattgattgcagctgagtagcaaggatggttcttaaggaagggaaagtgttccaagctttaggaattcaaggtttagtcaggtgtagcaattctattttattaggaggaatactatttctaatggcacttagcttttcacagcccttgtggatgcctaagaaagtgaaattaatcccatgccctcaagtgtgcagattggtcacagcatttcaagggagagacctcattgtaagactctgggggaggtggggacttaggtgtaagaaatgaatcagcagaggctcacaagtcagcatgagcatgttatgtctgagaaacagaccagcactgtgagatcaaaatgtagtgggaagaatttgtacaacattaattggaaggcttacttaatggaatttttgtatagttggatgttagtgcatctctataagtaagagtttaatatgatggtgttacggacctaatgtttgtgtctcctcaaaattcacatgctgaatccccaactcccaactgaccttatctgtgggggaggcttttgaaaagtaattaggtttagatgagctcataagagcagatccccatcataaaattattttccttatcagaagcagagagacaagccatttctctttcctcccggtgaggacacagtgagaagtccgccatctgcaatccaggaagagaaccctgaccacgagtcagccttcagaaatgtgagaaaaaactctgttgttgaagccacccagtcttttgtattttgttatagcaccttgcactgagtaaggcagatgaagaaggagaaaaaaataagcttgggttttgagtggactacagaccatgtttatctcaggtttgcaaagctcccctcgtcccctatgtttcagtataaaatacctactctactactctcatctataagacccaaataataagcctgcgcccttctctctaactttgatttctcctatttttacttcaacatgctttactctagccttgtaatgtctttacatacagtgaaatgtaaagttctttattctttttttctttctttcttttttctcctcagcctcagaatttggcacatgcccttccttctttcaggaacttctccaacatctctgcctggctccatcatatcataaaggtcccacttcaaatgcagtcactaccgtttcagaatatgcactttctttcttttttgttttttgttttttttaagtcaaagcaaatttcttgagagagtaaagaaataaacgaatgactactgcataggcagagcagccccgagggccgctggttgttccttttatggttatttcttgatgatatgttaaacaagttttggattatttatgccttctctttttaggccatatagggtaactttctgacattgccatggcatttttcttttaatttaatttactgttaccttaaattcaggggtacacgtacaggatatgcaggtttgttttataggtaaaagtgtgccatggttttaatgggttttttttttcttgtaaagttgtttaagtttcttgtttactctggatattaggcctttgtcagaagaatagattggaaaatctttttcccattctgtagattgtctttcgctctgatggtagtttcttttgctgagcaggagctctttagtttaattagattccattggtcaatttttgcttttgctgcaattgcttttcacgctttcatcatgaaatctgtgcccgtgtttatatcatgaatagtattgccttgatttttttctaggctttttatagtttggggtttttcatttaagtctctaatccatctggagttaattttggataaggtataaggaaggagtccagtttcatttttcagcatatggctagccagttctcccccatcatttattaaattgaaaatcctttccccattgcttgcttttgtcaggtttctaaaagaccagatggttgtaggtacaatatgcagtttcttcaagtcatataataccatctgaaatctcttattaattcatttcttttagtatgtatgctggtctcctctgctcactatagtgagggcaccattagccagagaatctgtctgtctagttcatgtaagattctcagaattaagaaaaatggatggcatatgaatgaaacttcatggatgacatatggaatctaatatgtatttgttgaattaatgcataagatgcaacagagagaagttgacaactgcaatgataacctggtattgatgatataagagtctatagatcacagtagaagcaataatcatggaaaacaattggaaatggggaacagccacaaacaagaaagaatcaatacttccaggaaagtgactgcaggtcacttttcctggagcgggtgagagaaaagtggaagttagcagtaactgctgaattcctggttggctgatggaaagatggggcagctgttcactggtacgcagggttttagatgtatgtacctaaggatatgaggtatggcaatgaacagaaattcttttgggaatgagttttagggccattaaaggacatgacctgaagtttcctctgaggccagtccccacaactcaatataaatgtgtttcctgcatatagtcaaagttgccacttctttttcttcatatcatcgatctctgctcttaaagataatcttggttttgcctcaaactgtttgtcactacaaactttccccatgttcctaagtaaaacaggtaactgcctctcaactatatcaagtagactaaaatattgtgtctctaatatcagaaattcagctttaatatattgggtttaactctttgaaatttagagtctccttgaaatacacatgggggtgatttcctaaactttatttcttgtaaggatttatctcaggggtaacacacaaaccagcatcctgaacctctaagtatgaggacagtaagccttaagaatataaaataaactgttcttctctctgccggtggaagtgtgccctgtctattcctgaaattgcttgtttgagacgcatgagacgtgcagcacatgagacacgtgcagcagcctgtggaatattgtcagtgaagaatgtctttgcctgattagatataaagacaagttaaacacagcattagactatagatcaagcctgtgccagacacaaatgacctaatgcccagcacgggccacggaatctcctatcctcttgcttgaacagagcagcacacttctcccccaacactattagatgttctggcataattttgtagatatgtaggatttgacatggactattgttcaatgattcagaggaaatctcctttgttcagataagtacactgactactaaatggattaaaaaacacagtaataaaacccagttttccccttacttccctagtttgtttcttattctgctttcttccaagttgatgctggatagaggtgtttatttctattctaaaaagtgatgaaattggccgggcgcggtggctcacacctgtaatcccagcactttgggaggctgaggtgggcggatcacgaggtcaggagatcaagaccatcctggctaacatggtgaaaccccatctctactaaaaatacaaaaaattagccagagacagtggcgggtgcctgtagtcccagctactcgggaggctgaggcaggagaatggcgtgaacctgggaggcagagcttgcggtgagcagagatcgcgccactgcacactccagcctgggtgacaaagcgagactccatctcaaaaaaaaaaaaaaaaaaaagaaaaagaaagaaagaaagaaaaaaaaactgatgaaattgtgtattcaatgtagtctcaagagaattgaaaaccaagaaaggctgtggcttcttccacataaagcctggatgaataacaggataacacgttgttacattgtcacaactcctgatccaggaattgatggctaagatattcgtaattcttatccttttcagttgtaacttattcctatttgtcagcattcaggttattagcggctgctggcgaagtccttgagaaataaactgcacactggatggtgggggtagtgtaggaaaatggaggggaaggaagtaaagtttcaaattaagcctgaacagcaaagttcccctgagaaggccacctggattctatcagaaactcgaatgtccatcttgcaaaacttccttgcccaaaccccacccctggagtcacaacccacccttgaccaatagattcattttactgagggaggcaaagggctggtcaatagattcatttcactgggagaggcaaagggctgggggccagagaggagaagtaaaaagccacacatgaagcagcaatgcaggcatgcttctggctcatctgtgatcaccaggaaactcccagatctgacactgtagtgcatttcactgctgacaagaaggctgctgccaccagcctgtgaagcaaggttaaggtgagaaggctggaggtgagattctgggcaggtaggtactggaagccgggacaaggtgcagaaaggcagaaagtgtttctgaaagagggattagcccgttgtcttacatagtctgactttgcacctgctctgtgattatgactatcccacagtctcctggttgtctacccatggacctagaggtactttgaaagttttggatatctgggctctgactgtgcaataatgggcaaccccaaagtcaaggcacatggcaagaaggtgctgatctccttcggaaaagctgttatgctcacggatgacctcaaaggcacctttgctacactgagtgacctgcactgtaacaagctgcacgtggaccctgagaacttcctggtgagtagtaagtacactcacgctttcttctttacccttagatatttgcactatgggtacttttgaaagcagaggtggctttctcttgtgttatgagtcagctatgggatatgatatttcagcagtgggattttgagagttatgttgctgtaaataacataactaaaatttggtagagcaaggactatgaataatggaaggccacttaccatttgatagctctgaaaaacacatcttataaaaaattctggccaaaatcaaactgagtgtttttggatgagggaacagaagttgagatagagaaaataacatctttcctttggtcagcgaaattttctataaaaattaatagtcacttttctgcatagtcctggaggttagaaaaagatcaactgaacaaagtagtgggaagctgttaaaaagaggattgtttccctccgaatgatgatggtatacttttgtacgcatggtacaggattctttgttatgagtgtttgggaaaattgtatgtatgtatgtatgtatgtatgtgatgactggggacttatcctatccattactgttccttgaagtactattatcctactttttaaaaggacgaagtctctaaaaaaaaaatgaaacaatcacaatatgttggggtagtgagttggcatagcaagtaagagaaggataggacacaatgggaggtgcagggctgccagtcatattgaagctgatatctagcccataatggtgagagttgctcaaactctggtgaaaaaggatgtaagtgttatatctatttactgcaagtccagcttgaggccttctattcactatgtaccattttcttttttatcttcactccctccccagctcttaggcaacgtgatattgattgttttggcaacccacttcagcgaggattttaccctacagatacaggcttcttggcagtaactaacaaatgctgtggttaatgctgtagcccacaagaccactgagttccctgtccactatgtttgtacctatggtccactatgtttgtacctatgtcccaaaatctcatctcctttagatgggggaggttggggagaagagcagtatcctgcctgctgattcagttcctgcatgataaaaatagaataaagaaatatgctctctaagaaatatcattgtactctttttctgtctttatattttaccctgattcagccaaaaggacgcactatttctgatggaaatgagaatgttggagaatgggagtttaaggacagagaagatactttcttgcaatcctgcaagaaaagagagaactcgtgggtggatttagtggggtagttactcctaggaaggggaaatcgtctctagaataagacaatgtttttacagaaagggaggtcaatggaggtactctttggaggtgtaagaggattgttggtagtgtgtagaggtatgttaggactcaaattagaagttctgtataggctattatttgtatgaaactcaggatatagctcatttggtgactgcagttcacttctacttattttaaacaacatattttttattatttataatgaagtggggatggggcttcctagagaccaatcaagggccaaaccttgaactttctcttaacgtcttcaatggtattaatagagaattatctctaaggcatgtgaactggctgtcttggttttcatctgtacttcatctgctacctctgtgacctgaaacatatttataattccattaagctgtgcatatgatagatttatcatatgtattttccttaaaggatttttgtaagaactaattgaattgatacctgtaaagtctttatcacactacccaataaataataaatctctttgttcagctctctgtttctataaatatgtacaagttttattgtttttagtggtagtgattttattctctttctatatatatacacacacatgtgtgcattcataaatatatacaatttttatgaataaaaaattattagcaatcaatattgaaaaccactgatttttgtttatgtgagcaaacagcagattaaaaggctgagatttaggaaacagcacgttaagtcaagttgatagaggagaatatggacatttaaaagaggcaggatgatataaaattagggaaactggatgcagagaccagatgaagtaagaaaaatagctatcgttttgagcaaaaatcactgaagtttcttgcatatgagagtgacataataaatagggaaacgtagaaaattgattcacatgtatatatatatatagaactgattagacaaagtctaacttgggtatagtcagaggagcttgctgtaattatattgaggtgatggataaagaactgaagttgatggaaacaatgaagttaagaaaaaaaatcgagtaagagaccattgtggcagtgattgcacagaactggaaaacattgtgaaacagagagtcagagatgacagctaaaatccctgtctgtgaatgaaaagaaggaaatttattgacagaacagcaaatgcctacaagccccctgtttggatctggcaatgaacgtagccattctgtggcaatcacttcaaactcctgtacccaagacccttaggaagtatgtagcaccctcaaacctaaaacctcaaagaaagaggttttagaagatataataccctttcttctccagtttcattaatcccaaaacctctttctcaaagtatttcctctatgtgtccaccccaaagagctcacctcaccatatctcttgagtgggagcacatagataggcggtgctaccatctaacagcttctgaaattcctttgtcatatttttgagtccccactaataacccacaaagcagaataaataccagttgctcatgtacaataatcactcaactgctgtcttgtagcatacattaattaagcacattctttgaataattactgtgtccaaacaatcacactttaaaatctcacacttgtgctatcccttgcccttctgaatgtcactctgtattttaaatgaagagatgagggttgaatttcctgtgttacttattgttcatttctcgatgaggagttttcacattcacctttagtggaaaacacataagtacacatcttacaggaaaaatataccaaactgacatgtagcatgaatgcttgtgcatgtagtcatataaaatcttgtagcaatgtaaacattctctgatatacacatacagatgtgtctatatgtctacacaatttcttatgctccatgaacaaacattccatgcacacataagaacacacactgttacagatgcatacttgagtgcattgacaaaattaccccagtcaatctagagaatttggatttctgcatttgactctgttagctttgtacatgctgttcatttactctgggtgatgtctttccctcattttgccttgtctatcttgtactcatactttaagtcctaacttatatgttatctcaactaagaagctatttttttttaattttaactgggcttaaagccctgtctataaactctgctacaattatgggctctttcttataatatttagtgtttttcctactaatgtacttaatctgctcattgtatattcctaccactaaattttaacctcttttatggtagagacattgtcttgtaaactcttatttccctagtatttggagatgaaaaaaaagattaaattatccaaaattagatctctcttttctacattatgagtattacactatccatagagaagtttgtttgagacctaaactgaggaacctttggttctaaaatgactatgtgatatcttagtatttataggtcatgaggttccttcctctgcctctgctatagtttgattagtcaacaagcatgtgtcatgcatttattcacatcagaatttcatacactaataagacatagtatcagaagtcagtttattagttatatcagttagggtccatcaaggaaaggacaaaccattatcagttactcaacctagaattaaatacagctcttaatagttaattatccttgtattggaagagctaaaatatcaaataaaggacagtgcagaaatctagatgttagtaacatcagaaaacctcttccgccattaggcctagaagggcagaaggagaaaatgtttataccaccagagtccagaaccagagcccataaccagaggtccactggattcagtgagctagtgggtgctccttggagagagccagaactgtctaatgggggcatcaaagtatcagccataaaaaaccataaaaaagactgtctgctgtaggagatccgttcagagagagagagagaccagaaataatcttgcttatgctttccctcagccagtgtttaccattgcagaatgtacatgcgactgaaagggtgaggaaacctgggaaatgtcagttcctcaaatacagagaacactgagggaaggatgagaaataaatgtgaaagcagacatgaatggtaattgacagaaggaaactaggatgtgtccagtaaatgaataattacagtgtgcagtgattattgcaatgattaatgtattgataagataatatgaaaacacagaattcaaacagcagtgaactgagattagaattgtggagagcactggcatttaagaatgtcacacttagaatgtgtctctaggcattgttctgtgcatatatcatctcaatattcattatctgaaaattatgaattaggtacaaagctcaaataatttattttttcaggttagcaagaactttttttttttttttctgagatagagcattgctatggttgcccaggctggagtgcaatggcatgatccaggctcactgcaacatctgcctcccaggttcaagcgattctcctgcctcagcctcccaagtagctggcactacaggcatgtgccaccaccatgcctggctaattttctatttttagtagatagggggtttcaccatgttggtcaggctgatctcgaactcctaacatcaggtgatccaccctcctcggcctctgaaagtgctgggatcacaggcgtgagccaccacacccagccaagaatgtgaattttgtagaaggatataacccatatttctctgaccctagagtccttagtatacctcccataccatgtggctcatcctccttacatacatttcccatctttcaccctaccttttcctttttgtttcagcttttcactgtgtcaaaatctagaaccttatctcctacctgctctgaaaccaacagcaagttgacttccattctaacccacattggcattacactaattaaaatcgatactgagttctaaaatcatcggggattttggggactatgtcttacttcatacttccttgagatttcacattaaatgttggtgttcattaaaggtccttcatttaactttgtattcatcacactcttggattcacagttatatctaaactcttaaatacagcctgtataatcccaattcccaactctgatttctaacctctgacctccaacctcagtgccaaacccatatatcaaacaatgtactgggcttatttatatagatgtcctataggcacctcagactcagcatgggtatttcacttgttatactaaaactgtttctcttccagtgttttccattttagtcattagatagctacttgcccattcaccaaggtcacagattaaaatcatttccctacctctaatcaacagttcgattctgcttcaatttgtccctatctattaatcaccactcttactgcccagtcaggtcctcattgtttcctgaacaagagtagatgctattctttccacttttagaccttatcctggctggatgcggtggctcaggcttgtaaacccagcactttgggaggccaaggcaggcagatcacttgaggtcaggagttcaagaccagcctgaccaacatggtgaaaccccatctctactaaaaatacaaaatcagccgggcgtgtggtgcatgcctgcagtcccagctattcaggtggctgaggcaggagaattgcttgaacccaggaggcagaggttgcggtgagcctagattgcaccattgcactctagcttgggcaatagggatgaaactccatctcagaagagaaaagaaaaaaagaccttattctgttatacaaatcctctcaatgcaatccatatagaataaacatgtaaccagatctcccaatgtgtaaaatcatttcaggtagaacagaattaaagtgaaaagccaagtctttggaattaacagacaaagatcaaataacagtcctcatggccttaagaatttacctaacattttttttagaatcaattttcttatatatgaattggaaacataattcctccctcacaaacacattctaagattttaaggagatattgatgaagtacatcatctgtcatttttaacaggtagtggtagtgattcacacagcacattatgatctgttcttgtatgttctgttccattctgtattcttgacctggttgtattctttctgagctccagatccacatatctaagtacatctttttgcattttacaagagtgcatacaatacaatgtatccaagactgtatttctgattttatcgtaccactaaactcacaaatgtggccctattcttgtgttcacgactgacatcaccgtcatggtccaagtctgataatagaaatggcattgtcactttcttccctactgcaacagaagcccagctatttgtctcccattttctctacttctaaaatacatttcttcactaagtgagaataatcttttaaagacacaaatcaaaccatgccaccacctttcttgaattattcaatatctttcgttggcttccaggttacagaaaaataacttgtaacaaagtttaaaggtcattcatggctcctctctaccctattttataacatttccccttgtgatcagaatctcaggcacatcatccatctttctatatacaaataaagtcatatagtttgaactcacctctggttacttttaatcaaccaaatgctgtaaaatgcatttgtatcgctacgtgttaagcagtagttgattcttttcatttctgtgtaatattctattctttgactataccgtaatttatcaattctactgttggtaagcatttaagtggctaccggtttgaggtttttatgattattgctgtcataagcatttctatacatgtctttggatacacacatgcatgtgtttctgaatatctaaaaatgtaattgctaggtaatagacttatcaagcatccagcatttgtggatactattaaaggttttccaaaggggttatactattgtacagtgtcaccaacagagtttgagtttctattgatccatatcaccaccaaaatttgaactgtcagtcttatctcttctcttgtctcttttttcctcttttttttccttcccttcccctctcttcgtttcttttctctcctcttctcttctttcctctcttcccttccctttctctttctcttccctatcccttctcctctcctctcccctccttttttctcctctcctctccattatttatttttccttcttctcctccatcccttccatcctctctcttcccctcttccttccttcctttctccatttcttcctcctctttccttcaatccttccttttggatatgctcatgggtgtgtatttgtctgccattgtggcattatttgaattcagaaaagagtgaaaaactactgggatcttcattcctgggtctaattccacatttttttttaagaacacatctgtaaaaatgttctgtactagcatattcccaggaacttcgttaaatttaatctggctgaatatggtaaatctacttttcactttgcattctttctttagtcataccataattttaaacattcaaaatatttgtatataatatttgattttatctgtcattaaaatgttaaccttaaaattcatgtttccagaacctatttcaataactggtaaataaacactattcattttttaaatattcttttaatggatatttatttcaatataataaaaaattagagttttattataggaagaatttaccaaaagaaggaggaagcaagcaagtttaaactgcagcaatagatttgtccattccaacctctcaaaattcccttggagacaaaaatctctagaggcaaagaagaactttatattgagtcaacttgttaaaacatctgcttttagataagttttcttagtataaagtgacagaaacaaataagttaaactctaagatacattccactatattagcctaaaacacttctgcaaaaatgaaactaggaggatatttttagaaacaactgctgaaagagatgcggtggggagatatgtagaggagaacagggtttctgagtcaagacacacatgacagaacagccaatctcagggcaagttaagggaatagtggaatgaaggttcatttttcattctcacaaactaatgaaaccctgcttatcttaaaccaacctgctcactggagcagggaggacaggaccagcataaaaggcagggcagagtcgactgttgcttacactttcttctgacataacagtgttcactagcaacctcaaacagacaccatggtgcatctgactcctgaggagaagactgctgtcaatgccctgtggggcaaagtgaacgtggatgcagttggtggtgaggccctgggcaggttggtatcaaggttataagagaggctcaaggaggcaaatggaaactgggcatgtgtagacagagaagactcttgggtttctgataggcactgactctctgtcccttgggctgttttcctaccctcagattactggtggtctacccttggacccagaggttctttgagtcctttggggatctgtcctctcctgatgctgttatgggcaaccctaaggtgaaggctcatggcaagaaggtgctaggtgcctttagtgatggcctggctcacctggacaacctcaagggcactttttctcagctgagtgagctgcactgtgacaagctgcacgtggatcctgagaacttcagggtgagtccaggagatgcttcacttttctctttttactttctaatcttacattttggttcttttacctacctgctcttctcccacatttttgtcattttactatattttatcatttaatgcttctaaaattttgttaattttttatttaaatattctgcattttttccttcctcacaatcttgctattttaaattatttaatatcctgtctttctctcccaaccccctcccttcatttttccttctctaacaacaactcaaattatgcataccagctctcacctgctaattctgcacttagaataatccttttgtctctccacatgggtatgggagaggctccaactcaaagatgagaggcatagaatactgttttagaggctataaatcattttacaataaggaataattggaattttataaattctgtagtaaatggaatggaaaggaaagtgaatatttgattatgaaagactaggcagttacactggaggtggggcagaagtcgttgctaggagacagcccatcatcacactgattaatcaattaatttgtatctattaatctgtttatagtaattaatttgtatatgctatatacacatacaaaattaaaactaatttggaattaatttgtatatagtattatacagcatatatagcatatatgtacatatatagactacatgctagttaagtacatagaggatgtgtgtgtatagatatatgttatatgtatgcattcatatatgtacttatttatgctgatgggaataacctggggatcagttttgtctaagatttgggcagaaaaaaatgggtgttggctcagtttctcagaagccagtctttatttctctgttaaccatatgcatgtatctgcctacctcttctccgcagctcttgggcaatgtgctggtgtgtgtgctggcccgcaactttggcaaggaattcaccccacaaatgcaggctgcctatcagaaggtggtggctggtgtggctaatgccctggctcacaagtaccattgagatcctggactgtttcctgataaccataagaagaccctatttccctagattctattttctgaacttgggaacacaatgcctacttcaagggtatggcttctgcctaataaagaatgttcagctcaacttcctgattaatttcacttatttcatttttttgtccaggtgtgtaagaaggttcctgaggctctacagatagggagcacttgtttattttacaaagagtacatgggaaaagagaaaagcaagggaaccgtacaaggcattaatgggtgacacttctacctccaaagagcagaaattatcaagaactcttgatacaaagataatactggcactgcagaggttctagggaagacctcaaccctaagacatagcctcaagggtaatgctacgattaaactccaacaattactgagaaaataatgtgctcaattaaaggcataatgattactcaagacaatgttatgttgtctttcttcctccttcctttgcctgcacattgtagcccataatactataccccatcaagtgttcctgctccaagaaatagcttcctcctcttacttgccccagaacatctctgtaaagaatttcctcttatcttcccatatttcagtcaagattcattgctcacgtattacttgtgacctctcttgaccccagccacaataaacttctctatactacccaaaaaatctttccaaaccctcccccacaccattttttatatttttatatttttcttatttatttcatgcacacacacacactccgtgctttataagcaattctgcctattctctaccttcttacatgcctactgtgcctcatattaaattcatcaatgggcagaaagaaaatatttattcaagaaaacagtgaatgaatgaacgaatgagtaaatgagtaaatgaaggaatgattattccttgctttagaacttctggaattagaggacaatattaataataccatcgcacagtgtttctttgttgttaatgctacaacatacaaagaggaagcatgcagtaaacaaccgaacagttatttcctttctgatcataggagtaatatttttttccttgagcaccatttttgccataggtaaaattagaaggatttttagaactttctcagttgtatacatttttaaaaatctgtattatatgcatgttgattaattttaaacttacttgaatacctaaacagaatctgttgtttccttgtgtttgaaagtgctttcacagtaactctgtctgtactgccagaatatactgacaatgtgttatagttaactgttttgatcacaacattttgaattgactggcagcagaagctcttttatatccatgtgttttccttaagtcattatacatagtaggcactgagaactctttatatctgaataagatatttaggaaccactggtttacatatcagaagcagagctactcagggcattttggggaagatcactttcacattcctgagcatagggaagttctcataagagtaagatattaaaaggagatacttgtgtggtattcgaaagacagtaagagagattgtagaccttatgatcttgatagggaaaacaaactacattcctttctccaaaagtcaaaaaaaaagagcaaatatagcttactataccttctattcctacaccattagaagtagtcagtgagtctaggcaagatgttggccctaaaaatccaaataccagagaattcatgagaacatcacctggatgggacatgtgccgagcacacacaattactatatgctaggcattgctatcttcatattgaagatgaggaggtcaagagatgaaaaaagacttggcaccttgttgttatattaaaattatttgttagagtagagcttttgtaagagtctaggagtgtgggagctaaatgatgatacacatggacacaaaaaatagatcaacagacacccaggcctacttgagggttgagggtgggaagagggagacgatgaaaaagaacctattgggtattaagttcatcactgagtgatgaaataatctgtacatcaagacccagtgatatgcaatttacctatataacttgtacatgtacccccaaatttaaaatgaaagttaaaacaaagtataggaatggaattaattcctcaagatttggctttaattttatttgataatttatcaaatggttgtttttcttttctcactatggcgttgctttataaactatgttcagtatgtctgaatgaaagggtgtgtgtgtgtgtgaaagagagggagagaggaagggaagagaggacgtaataatgtgaatttgagttcatgaaaatttttcaataaaataatttaatgtcaggagaattaagcctaatagtctcctaaatcatccatctcttgagcttcagagcagtcctctgaattaatgcctacatgtttgtaaagggtgttcagactgaagccaagattctacctctaaagagatgcaatctcaaatttatctgaagactgtacctctgctctccataaattgacaccatggcccacttaatgaggttaaaaaaaagctaattctgaatgaaaatctgagcccagtggaggaaatattaatgaacaaggtgcagactgaaatataaatttttctgtaataattatgcatatactttagcaaagttctgtctatgttgactttattgctttttggtaagaaatacaactttttaaagtgaactaaactatcctatttccaaactattttgtgtgtgtgcggtttgtttctatgggttctggttttcttggagcatttttatttcattttaattaattaattctgagagctgctgagttgtgtttactgagagattgtgtatctgcgagagaagtctgtagcaagtagctagactgtgcttgacctaggaacatatacagtagattgctaaaatgtctcacttggggaattttagactaaacagtagagcatgtataaaaatactctagtcaagtgctgcttttgaaacaaatgataaaaccacactcccatagatgagtgtcatgattttcatggaggaagttaatattcatcctctaagtatacccagactagggccattctgatataaaacattaggacttaagaaagattaatagactggagtaaaggaaatggacctctgtctctctcgctgtctcttttttgaggacttgtgtgtgtgtgtgtgtgtgtgtgtgtgtgtgtgttgtggtcagtggggctggaataaaagtagaatagacctgcacctgctgtggcatccattcacagagtagaagcaagctcacaatagtgaagatgtcagtaagcttgaatagtttttcaggaactttgaatgctgatttagatttgaaactgaggctctgaccataaccaaatttgcactatttattgcttcttgaaacttatttgcctggtatgcctgggcttttgatggtcttagtatagcttgcagccttgtccctgcagggtattatgggtaatagaaagaaaagtctgcgttacactctagtcacactaagtaactaccattggaaaagcaacccctgccttgaagccaggatgatggtatctgcagcagttgccaacacaagagaaggatccatagttcatcatttaaaaaagaaaacaaaatagaaaaaggaaaactatttctgagcataagaagttgtagggtaagtctttaagaaggtgacaatttctgccaatcaggatttcaaagctcttgctttgacaattttggtctttcagaatactataaatataacctatattataatttcataaagtctgtgcattttctttgacccaggatatttgcaaaagacatattcaaacttccgcagaacactttatttcacatatacatgcctcttatatcagggatgtgaaacagggtcttgaaaactgtctaaatctaaaacaatgctaatgcaggtttaaatttaataaaataaaatccaaaatctaacagccaagtcaaatctgcatgttttaacatttaaaatattttaaagacgtcttttcccaggattcaacatgtgaaatcttttctcagggatacacgtgtgcctagatcctcattgctttagttttttacagaggaatgaatataaaaagaaaatacttaaattttatccctcttacctctataatcatacataggcataattttttaacctaggctccagatagccatagaagaaccaaacactttctgcgtgtgtgagaataatcagagtgagattttttcacaagtacctgatgagggttgagacaggtagaaaaagtgagagatctctatttatttagcaataatagagaaagcatttaagagaataaagcaatggaaataagaaatttgtaaatttccttctgataactagaaatagaggatccagtttcttttggttaacctaaattttatttcattttattgttttattttattttattttattttattttgtgtaatcgtagtttcagagtgttagagctgaaaggaagaagtaggagaaacatgcaaagtaaaagtataacactttccttactaaaccgacatgggtttccaggtaggggcaggattcaggatgactgacagggcccttagggaacactgagaccctacgctgacctcataaatgcttgctacctttgctgttttaattacatcttttaatagcaggaagcagaactctgcacttcaaaagtttttcctcacctgaggagttaatttagtacaaggggaaaaagtacagggggatgggagaaaggcgatcacgttgggaagctatagagaaagaagagtaaattttagtaaaggaggtttaaacaaacaaaatataaagagaaataggaacttgaatcaaggaaatgattttaaaacgcagtattcttagtggactagaggaaaaaaataatctgagccaagtagaagaccttttcccctcctacccctactttctaagtcacagaggctttttgttcccccagacactcttgcagattagtccaggcagaaacagttagatgtccccagttaacctcctatttgacaccactgattaccccattgatagtcacactttgggttgtaagtgactttttatttatttgtatttttgactgcattaagaggtctctagttttttatctcttgtttcccaaaacctaataagtaactaatgcacagagcacattgatttgtatttattctatttttagacataatttattagcatgcatgagcaaattaagaaaaacaacaacaaatgaatgcatatatatgtatatgtatgtgtgtatatatacacacatatatatatatattttttcttttcttaccagaaggttttaatccaaataaggagaagatatgcttagaaccgaggtagagttttcatccattctgtcctgtaagtattttgcatattctggagacgcaggaagagatccatctacatatcccaaagctgaattatggtagacaaaactcttccacttttagtgcatcaacttcttatttgtgtaataagaaaattgggaaaacgatcttcaatatgcttaccaagctgtgattccaaatattacgtaaatacacttgcaaaggaggatgtttttagtagcaatttgtactgatggtatggggccaagagatatatcttagagggagggctgagggtttgaagtccaactcctaagccagtgccagaagagccaaggacaggtacggctgtcatcacttagacctcaccctgtggagccacaccctagggttggccaatctactcccaggagcagggagggcaggagccagggctgggcataaaagtcagggcagagccatctattgcttacatttgcttctgacacaactgtgttcactagcaacctcaaacagacaccatggtgcatctgactcctgaggagaagtctgccgttactgccctgtggggcaaggtgaacgtggatgaagttggtggtgaggccctgggcaggttggtatcaaggttacaagacaggtttaaggagaccaatagaaactgggcatgtggagacagagaagactcttgggtttctgataggcactgactctctctgcctattggtctattttcccacccttaggctgctggtggtctacccttggacccagaggttctttgagtcctttggggatctgtccactcctgatgctgttatgggcaaccctaaggtgaaggctcatggcaagaaagtgctcggtgcctttagtgatggcctggctcacctggacaacctcaagggcacctttgccacactgagtgagctgcactgtgacaagctgcacgtggatcctgagaacttcagggtgagtctatgggacgcttgatgttttctttccccttcttttctatggttaagttcatgtcataggaaggggataagtaacagggtacagtttagaatgggaaacagacgaatgattgcatcagtgtggaagtctcaggatcgttttagtttcttttatttgctgttcataacaattgttttcttttgtttaattcttgctttctttttttttcttctccgcaatttttactattatacttaatgccttaacattgtgtataacaaaaggaaatatctctgagatacattaagtaacttaaaaaaaaactttacacagtctgcctagtacattactatttggaatatatgtgtgcttatttgcatattcataatctccctactttattttcttttatttttaattgatacataatcattatacatatttatgggttaaagtgtaatgttttaatatgtgtacacatattgaccaaatcagggtaattttgcatttgtaattttaaaaaatgctttcttcttttaatatacttttttgtttatcttatttctaatactttccctaatctctttctttcagggcaataatgatacaatgtatcatgcctctttgcaccattctaaagaataacagtgataatttctgggttaaggcaatagcaatatctctgcatataaatatttctgcatataaattgtaactgatgtaagaggtttcatattgctaatagcagctacaatccagctaccattctgcttttattttatggttgggataaggctggattattctgagtccaagctaggcccttttgctaatcatgttcatacctcttatcttcctcccacagctcctgggcaacgtgctggtctgtgtgctggcccatcactttggcaaagaattcaccccaccagtgcaggctgcctatcagaaagtggtggctggtgtggctaatgccctggcccacaagtatcactaagctcgctttcttgctgtccaatttctattaaaggttcctttgttccctaagtccaactactaaactgggggatattatgaagggccttgagcatctggattctgcctaataaaaaacatttattttcattgcaatgatgtatttaaattatttctgaatattttactaaaaagggaatgtgggaggtcagtgcatttaaaacataaagaaatgaagagctagttcaaaccttgggaaaatacactatatcttaaactccatgaaagaaggtgaggctgcaaacagctaatgcacattggcaacagcccctgatgcatatgccttattcatccctcagaaaaggattcaagtagaggcttgatttggaggttaaagttttgctatgctgtattttacattacttattgttttagctgtcctcatgaatgtcttttcactacccatttgcttatcctgcatctctcagccttgactccactcagttctcttgcttagagataccacctttcccctgaagtgttccttccatgttttacggcgagatggtttctcctcgcctggccactcagccttagttgtctctgttgtcttatagaggtctacttgaagaaggaaaaacaggggtcatggtttgactgtcctgtgagcccttcttccctgcctcccccactcacagtgacccggaatctgcagtgctagtctcccggaactatcactctttcacagtctgctttggaaggactgggcttagtatgaaaagttaggactgagaagaatttgaaaggcggctttttgtagcttgatattcactactgtcttattaccctgtcataggcccaccccaaatggaagtcccattcttcctcaggatgtttaagattagcattcaggaagagatcagaggtctgctggctcccttatcatgtcccttatggtgcttctggctctgcagttattagcatagtgttaccatcaaccaccttaacttcatttttcttattcaatacctaggtaggtagatgctagattctggaaataaaatatgagtctcaagtggtccttgtcctctctcccagtcaaattctgaatctagttggcaagattctgaaatcaaggcatataatcagtaataagtgatgatagaagggtatatagaagaattttattatatgagagggtgaaaccctcaaaatgaaatgaaatcagacccttgtcttacaccataaacaaaaataaatttgaatgggttaaagaattaaactaagacctaaaaccataaaaatttttaaagaaatcaaaagaagaaaattctaatattcacgttgcagccgttttttgaatttgatatgagaagcaaaggcaacaaaaggaaaaataaagaagtgaggctacatcaaactaaaaaatttccacacaaaaaacaaaacaatgaacaaatgaaaggtgaaccatgaaatggcatatttgcaaaccaaatatttcttaaatattttggttaatatccaaaatatataagaaacacagatgattcaataacaaacaaaaaattaaaaataggaaaataaaaaaattaaaaagaagaaaatcctgccatttatggcagaattgatgaacctggaggatgtaaaactaagaaaaataagcctgacacaaaaagacaaatactacacaaccttgctcatatgtgaaacataaaaaagtcactctcatggaaacagacagtagaggtatggtttccaggggttgggggtgggagaatcaggaaactattactcaaagggtataaaatttcagttatgtgggatgaataaattctagatatctaatgtacagcatcgtgactgtagttaattgtactgtaagtatatttaaaatttgcaaagagagtagatttttttttttttttagatggagttttgctcttgttgtccaggctggagtgcaatggcaagatcttggctcactgcaacctccgcctcctgggttcaagcaaatctcctgcctcagcctcccgagtagctgggattacaggcatgcgacaccatgcccagctaattttgtatttttagtagagacggggtttctccatgttggtcaggctgatccgcctgcctcggccacccaaagggctgggattacaggcgtgagccaccgggcctggccgagagtagatcttaaaagcatttaccacaagaaaaaggtaactatgtgagataatgggtatgttaattagcttgattgtggtaatcatttcacaaggtatacatatattaaaacatcatgttgtacaccttaaatatatacaatttttatttgtgaatgatacctcaataaagttgaagaataataaaaaagaatagacatcacatgaattaaaaaactaaaaaataaaaaaatgcatcttgatgattagaattgcattcttgatttttcagatacaaatatccatttgactgtttactcttttccaaaacaatacaataaattttagcactttatcttcattttccccttcccaatctataattatatatatatatattttagatattttgtatagttttactccctagattttctagtgttattattaaatagtgaagaaatgtttacacttatgtacaaaatgttttgcatgcttttcttcatttctaacattctctctaagtttattctatttttttctgattatccttaatattatctctttctgctggaaatacattgttacttttggtttatctaaaaatggcttcattttcttcattctaaaatcatgttaaattaataccactcatgtgtaagtaagatagtggaataaatagaaatccaaaaactaaatctcactaaaatataataatgtgatatataaaaatatagcttttaaatttagcttggaaataaaaaacaaacagtaattgaacaactatactttttgaaaagagtaaagtgaaatgcttaactgcatataccacaatcgattacacaattaggtgtgaaggtaaaattcagtcacgaaaaaactagaataaaaatatgggaagacatgtatataatcttagagataacactgttatttaattatcaacccaaagtagaaactatcaagggagaaataaattcagtcaacaataaaagcatttaagaagttattctaggctgggagcggtggctcacacctgcaattgcagcactttgggaggcctagacaggcggatcacgacgtcaggagttcaagatcagcctggccaacatagtgaaacctcatcgctactaaaaatataaaaacttagcctggcgtggtggcaggcatgtgtaatcccagcaatttgggaggctgaggcaggagaatcgcttgatcctgggaggcagaggttgcagtgagccaagattgtgccactgcattccagcccaggtgacagcatgagactccgtcacaaaaaaaaaagaaaaaaaaaaggggggggggagcggtggagccaagatgaccgaataggaacagctccagtctatagctcccatcgtgagtgacgcagaagacgggtgatttctgcatttccaactgaggtaccaggttcatctcacagggaagtgccaggcagtgggtgcaggacagtaggtgcagtgcactgtgcatgagccaaagcagggcgaggcatcacctcacccgggaagcacaaggggtcagggaattccctttcctagtcaaagaaaagggtgacagatggcacctggaaaatcgggtcactcccgccctaatactgcgctcttccaacaagcttaacaaatggcacaccaggagattatatcccatgcctggctcagagggtcctacgcccatggagcctcgctcattgctagcacagcagtctgaggtcaaactgcaaggtggcagtgaggctgggggaggggtgcccaccattgtccaggcttgagcaggtaaacaaagccgcctggaagctcgaactgggtggagcccaccacagctcaaggaggcctgcctgcctctgtaggctccacctctaggggcagggcacagacaaacaaaagacaacaagaacctctgcagacttaaatgtccctgtctgacagctttgaagagagtagtggttctcccagcacatagcttcagatctgagaacaggcagactgcctcctcaagtgggtccctgacccccgagtagcctaactgggaggcatcccccagtaggggcagactgacacctcacatggctggtactcctctaagacaaaacttccagaggaatgatcaggcagcagcatttgcggttcaccaatatccactgttctgcagccaccgctgttgatacccaggaaaacagcttctggagtggacctccagtaaactccaacagacctgcagctgagggtcctgactgttagaaggaaaactaacaaacagaaaggacatccacaccaaaaacccatctgtacatcgccatcatcaaagaccaaaggtagataaaaccataaagatggggaaaaagcagagcagaaaaactggacactctaaaaatgagagtgcctctcctcctccaaagtaacgcagctcctcaccagcaatggaacaaagctgggcagagaatgactttgacgagttgagagaggaaggcttcagaagatcaaactactccaagctaaaggaggaagttcgaacaaacggcaaagaagtaaaaaactttgaaaaaaaattagatgaatggataactagaataaccaatgcacagaagtccttaaaggacctgatggagctgaaaaccaaggcaggagaactacgtgacaaatacacaagcctcagtaaccgatgagatcaactggaagaaagggtatcaatgacgaaagatgaaatgaatgaaatgaagcatgaagagaagtttagagaaaaaagaataaaaagaaacgaacaaagcctccaagaaatatgggactatgtgaaaagaccaaatctacatctaattggtgtagctgaaagtgatggggagaatggaaccaagttggaaaacactctgcaggatattatccaggagaacttccccaatctagcaaggcaagcccaaattcacattcaggaaatacagagaacgccacaaagatactcctagagaaaagcaactccaagacacataactgtcagattcaccaaagttgaaatgaaggaaaaaatgttaagggcagccagagagaaaggtcgggttacccacaaagggaagcccatcagactaacagctgatctatcggcagaaactctacaagccagaagaaagtgggggccaatattcaacattgttaaagaaaagaattttcaacccagaatttcatatccagccaaactaagcttcataagtgaaggagaaataaaatcctttacagacaagcaaatgctgagagattttgtcaccaccaggcctgccctacaagagctcctgaaggaagcactaaacatggaaaggaacaactagtatcagccactgcaaaaacatgccaaattgtaaagaccatcaaggctaggaagaaactgcatcaacgagcaaaataaccagctaacatcataatgacaggatcaaattcatacataacaatactcaccttaaatgtaaataggctaaatgctccaattaaaagacacagactggcaaattggataaggagtcaagacccatctgtgttctgtattcaggaaacccatctcacgtgcagagacacacataggctcgaaataaaaggatggaggaatatctaccaagcaaatggaaaacaaaaaaaggcaggggttgcaatcctagtctctgataaaacagattttaaaccaacaaagatcaaaagagacaaagaaggccattacataatggcaaagggatctattcaagaagaagaactaactatactaaatatatatgcacccaatacaggagcacccagattcataaaacaagtcctgagtgacctacaaagagacttagatgcccacacaataataatgggagactttaacaccccactgtcaacattagacagatcaacgagacagaaagttaacaaggatatccaggaattggactcagctctgcaccaagcagacctaatagacatctacagaactctccaccccaaatcaacagaatatacattcttttcagcaccacaccacacctattccaaaactgaccacatagttggaagtaaagctctcctcagcaaatgtaaaagaacagaaactataacaaactgtctctcagaccacagtgcaatcaaactagaactcaggattaagaaactcactcaaaaccactcagctacatggaaactgaacagcctgctcctgaatgactactgggtacataacaaaatgaaggcagaaataaagatgttctttgaaaccaacgagaacaaagacacaacacaccagaatctctgagacacattcaaagcagtgtgtagagggaaatttatagcactaaatgcccacaagggaaagcaggaaagatctaaaattgacaccctaacatcacaattaaaaaactagagaagcaggagcaaacacattcaaaagctaacagaagacaagaaataactaagatcagagcagaagtgaaggacatagagacacaaaaaaacccttcaaaaaaatcaatgaatccagaagctgtttttttgaaaagatcaacaaaattgatagactgctagcaagactaataaagaagaaaagagagaagaatcaaatagacgcaataaaaaatgacacggggtatcaccactgatcccacagaaatacaaactaccgtcagagaatactataaacacctctacgcaaataaactagaaaatctagaagaaatggataaattcctcgacacatacactctgccaagactaaaccaggaagaagttgtatctctgaatagaccaataacaggctctgaaattgaggcaataattaatagcttatcaaccaaaaaaagtccgggaccagtaggattcatagccgaattctaccagaggtacaaggaggagctggtaccattccttctgaaactattccaatcaatagaaaaagagggaatcctccctaactcattttatgaggccagcatcatcctgataccaaagcctgacagagacacaacaaaaaaagagaatgttacaccaatatccttgatgaacattgatgcaaaaatcctcaataaaatactggcaaactgatccaccatgatcaagtgggcttcatccctgccatgcaaggctggttcaacatacgaaaatcaataaacataatccagcatataaacagaaccaaagacacaaaccatatgattatctcaatagatgcagaaaaggcctttgacaaaattcaacaacgcttcatgctaaaaactctcaataaattaggtattgatgggacatatctcaaaataataagagctatctatgacaaacccacagccaatatcatactgagtggacaaaaactggaagcattccctttgaaaactggcacaaggcagggatgccctctctcaccactcctattcaacatagtgttgtaagttctggccagggcaatcaggcaggagaaggaaataaagggcattcaattaggaaaagaggaagtgaaattgtccctgtttgcagatgacatgattgtatatctagaaaaccccattgtctcagcccaaaatctccttaagctgataagcaacttcagcaaagtctcaggatataaaatcagtgtgcaaaaatcacaagtattcctatgcaccaataacagacaaacagagagccaaatcatgagtgaactcccattcacaattgcttcaaagagaataaaatacctaggaatccaacttacaagggatgtgaaggacctcttcaaggagaactacaaaccactgctcaatgaaataaaagaggatacaaacaaatggaagaacattccatgctcatgggtaggaagaatcaatatcgtgaaaatggtcatactgcccaaggtaatttatagattcaatgccatccccatcaagctaccaatgactttcttcacagaactggaaaaaactactttaaagttcatatggaaccaaaaaagagcccacatcaccaaggcaatcctaagccaaaagaacaaagctggaggcatcacgctacctgacttcaaactatactacaatgctacggtaaccaaaacagcatggtactggtaccaaaacagagatctagaccaatggaacagaacagagccctcagaaataatgccgcatatctacaactatctgatctttgacaaacctgagagaaacaagcaatggggaaaggattccctatttaataaatggtgctgggaaaactggctagccatatgtagaaagctgaaactggatcccttccttacaccttatacaaaaattaattcaagatggattaaagacttacatgttagacctaaaaccataaaaaccctagaaaaaaacctaggcaataccattcaggacataggcatgggcaaggacttcatgtctaaaacaccaaaagcaatggcaacaaaagacaaaatggacaaacgggatctaattaaactaaagagcttctgcacagctaaagaaactaccatcagagtgaacaggcaacctacaaaatgggagaaaatttttgcaatctactcatctgacaaagggctaatatccagaatctacaatgaactcaaacaaatttacaagaaaaaacaaacaaccccatcaaaaagtgggcaaaggatatgaacagacacttcgcaaaagaagacatttatgtaatcaaaaaacacatgaaaaaatgctcatcatcactagccatcagagaaatgcaaatcaaaaccacaatgagataccatctcacaccagttagaatggcgatcattaaaaagtcaggaaacaacaggtgctggagaggatgtggagaaacaggaacaacttttacactgttggtgggactgtaaactagttcaaccattgcggaagtcagtgtggcaattcctcaggaatctagaactagaaataccatttgacccagccatcccattactgggtacatacccaaaggattataaatcatgctgctataaagacacatgcacacgtatgtttattgcagcactattcacaatagcaaagacttggaaccaacccaaatgtccaacaacgatagactggattaagaaaatgtggcacatatacaccatggaatactatgcagccataaaaaatgatgagttcatgtcctttgtagggacatggatgaagctggaaactatcattctcagcaaactatcacaaggagaataaaccaaacaccgcatgttctcactcataggtgggaattgaacaatgagaacacatggacacatgaagaggaacatcacactctggggactgttatggggtggggggcaggggcagggatagcactaggagatatacctaatgctaaatgacgagttaatgggtgcagcacaccaacatggcacatgtatacatatataacaaacctgcatgttgtgcacatgtaccctaaaacttgaagtataataataaaaaaaagttatcctattaaaactgatctcacacatccgtagagccattatcaagtctttctctttgaaatagacagaaatttagtgttttctcagtcagttaac

SEQ ID NO: 20 - DNA, 388 bp, Homo sapiens
taagcttcagtttttccttagttcctgttacatttctgtgtgtctccattagtgacctcccatagtccaagcatgagcagttctggccaggcccctgtcggggtcagtgccccacccccgccttctggttctgtgtaaccttctaagcaaaccttctggctcaagcacagcaatgctgagtcatgatgagtcatgctgaggcttagggtgtgtgcccagatgttctcagcctagagtgatgactcctatctgggtccccagcaggatgcttacagggcagatggcaaaaaaaaggagaagctgaccacctgactaaaactccacctcaaacggcatcataaagaaaatggatgcctgagacagaatgtgacatattctagaatatatt

SEQ ID NO: 21 - DNA, 387 bp, Homo sapiens
taagcttcagtttttccttagttcctgttacatttctgtgtgtctccattagtgacctcccatagtccaagcatgagcagttctggccaggcccctgtcggggtcagtgccccacccccgccttctggttctgtgtaaccttctaagcaaaccttctggctcaagcacagcaatgctgagtcatgatgagtcatgctgaggctagggtgtgtgcccagatgttctcagcctagagtgatgactcctatctgggtccccagcaggatgcttacagggcagatggcaaaaaaaaggagaagctgaccacctgactaaaactccacctcaaacggcatcataaagaaaatggatgcctgagacagaatgtgacatattctagaatatatt

SEQ ID NO: 22 - DNA, 286 bp, Homo sapiens
ctgagcaactaactcatgcaggactctcaaacactaacctatagccttttctatgtatctacttgtgtagaaaccaagcgtggggactgagaaggcaatagcaggagcattctgactctcactgcctttggctaggtccctccctcatcacagctcagcatagtccgagctcttatctatatccacacacagtttctgacgctgcccagctatcaccatcccaagtctaaagaaaaaaataatgggtttgcccatctctgttgattagaaaacaaaacaaaataaa

SEQ ID NO: 23 - DNA, 286 bp, Homo sapiens
ctgagcaactaatcatgcaggactctcaaacactaacctatagccttttctatgtatctacttgtgtagaaaccaagcgtggggactgagaaggcaatagcaggagcattctgactctcactgcctttagctaggcccctccctcatcacagctcagcatagtcctgagctcttatctatatccacacacagtttctgacgctgcccagctatcaccatcccaagtctaaagaaaaaaataatgggtttgcccatctctgttgattagaaaacaaaacaaaataaa

SEQ ID NO: 24 - DNA, 301 bp, Homo sapiens
ccaatcgtggcatatcctctaaactttcttttcccttcataaatcctctttcttttttttccccctcacagttttcctgaacaggttgactattaattgtgtctgcttgatgtggacaccaggtggcgctggacatcagatttggagaggcagttgtctagggaaccgggctctgtgccagcgcaggaggcaggctggctctcctattccagggatgctcatccaggaaggaaaggttgcatgctggacacactaaccttgaagaattcttctgtctctctcgtcatttagaaaggaagga

SEQ ID NO: 25 - DNA, 305 bp, Homo sapiens
ctagccaatcgtggcatatcctctaaactttcttttcccttcataaatcctctttcttttttttccccctcacagttttcctgaacaggttgactattaattgtgtctgcttgatgtggacaccaggtggcgctggacatcagatttggagaggcagttgtctagggaaccgggctctgtgccagcgcaggaggcaggctggctctcctactccagggatgctcatccaggaaggaaaggttgcatgctggacacactaaccttgaagaattcttctgtctctctcgtcatttagaaaggaagga

SEQ ID NO: 26 - DNA, 896 bp, Artificial Sequence
  Description of Artificial Sequence: Synthetic polynucleotide
ctcgagttaattaatctcccacgccctggtctcagcttggggagtggtcagaccccaatggcgataaactctggcaactttatctgtgcactgcaggctcagccccaacagctttagctttcacaagcaggcaggggaagggaaacacatatctccagatatgaggttaattaacctgcaggctaaacccctcccccaccctagccccaagcttcatcttagctccactcctgaccctatccagctaaaggtccccacccagctcctgcctatctagtcattgcatatggcaagacttgaaagtcctatctcaaagcagcagaattatcagctacgactcctgcaggttataaccatcccccagcactccctgcccccacagcccagacttgaccaactcccagctccgcctgggacttccagatatggggccccacccttgcaggccttggggacgctgaagatattgactatctgcgtgccggaaaagggtgttataaaccggtaaaggctgggggtgggagtagcggatttgaagcacttgttggcctacagaggtgtggcaagcagagcacctcagaactcaggcgtactgcccgccgcccgagccctgcgagggccgatagcgagggtgtggcccttatctgcacccagcagagcgccggcggggtacggtcaccggtcccgggcagttgcctcagctgagtatgtcttctaaagataatgtcgattgtgtatggctgatgggattctaggaccaagcaagaggtttttttttttcccccacatacttaacgtttctatatttctatttgaattcgactggacagttccatttgaattatttctctctctctctctctctgacacattttatcttgccacccgggctcgag